European Patent Specification EP 3 611 261 B1, published June 24, 2026. Title: A method for designing RNA binding protein using PPR motif and a use thereof. Applicant: Kyushu University. The sequence listing filed with the application follows.

SEQUENCE LISTING (591 sequences)

SEQ ID NO: 1 - protein, 555 aa, Arabidopsis thaliana
MLRHAIETNVQIFTKFLVISASAVGIGYARKLFDQRPQRDDSFLSNSMIKAYLETRQYPDSFALYRDLRKETCFAPDNFTFTTLTKSCSLSMCVYQGLQLHSQIWRFGFCADMYVSTGVVDMYAKFGKMGCARNAFDEMPHRSEVSWTALISGYIRCGELDLASKLFDQMPHVKDVVIYNAMMDGFVKSGDMTSARRLFDEMTHKTVITWTTMIHGYCNIKDIDAARKLFDAMPERNLVSWNTMIGGYCQNKQPQEGIRLFQEMQATTSLDPDDVTILSVLPAISDTGALSLGEWCHCFVQRKKLDKKVKVCTAILDMYSKCGEIEKAKRIFDEMPEKQVASWNAMIHGYALNGNARAALDLFVTMMIEEKPDEITMLAVITACNHGGLVEEGRKWFHVMREMGLNAKIEHYGCMVDLLGRAGSLKEAEDLITNMPFEPNGIILSSFLSACGQYKDIERAERILKKAVELEPQNDGNYVLLRNLYAADKRWDDFGMVKNVMRKNQAKKEVGCSLIEINYIVSEFISGDTTHPHRRSIHLVLGDLLMHMNEEKYNW

SEQ ID NO: 2 - protein, 500 aa, Arabidopsis thaliana
MGLLPVVGITSPALITHKNHANPKIQRHNQSTSETTVSWTSRINLLTRNGRLAEAAKEFSDMTLAGVEPNHITFIALLSGCGDFTSGSEALGDLLHGYACKLGLDRNHVMVGTAIIGMYSKRGRFKKARLVFDYMEDKNSVTWNTMIDGYMRSGQVDNAAKMFDKMPERDLISWTAMINGFVKKGYQEEALLWFREMQISGVKPDYVAIIAALNACTNLGALSFGLWVHRYVLSQDFKNNVRVSNSLIDLYCRCGCVEFARQVFYNMEKRTVVSWNSVIVGFAANGNAHESLVYFRKMQEKGFKPDAVTFTGALTACSHVGLVEEGLRYFQIMKCDYRISPRIEHYGCLVDLYSRAGRLEDALKLVQSMPMKPNEVVIGSLLAACSNHGNNIVLAERLMKHLTDLNVKSHSNYVILSNMYAADGKWEGASKMRRKMKGLGLKKQPGFSSIEIDDCMHVFMAGDNAHVETTYIREVLELISSDLRLQGCVVETLAGDLLNA

SEQ ID NO: 3 - protein, 830 aa, Arabidopsis thaliana
MASLPFNTIPNKVPFSVSSKPSSKHHDEQAHSPSSTSYFHRVSSLCKNGEIKEALSLVTEMDFRNLRIGPEIYGEILQGCVYERDLSTGKQIHARILKNGDFYARNEYIETKLVIFYAKCDALEIAEVLFSKLRVRNVFSWAAIIGVKCRIGLCEGALMGFVEMLENEIFPDNFVVPNVCKACGALKWSRFGRGVHGYVVKSGLEDCVFVASSLADMYGKCGVLDDASKVFDEIPDRNAVAWNALMVGYVQNGKNEEAIRLFSDMRKQGVEPTRVTVSTCLSASANMGGVEEGKQSHAIAIVNGMELDNILGTSLLNFYCKVGLIEYAEMVFDRMFEKDVVTWNLIISGYVQQGLVEDAIYMCQLMRLEKLKYDCVTLATLMSAAARTENLKLGKEVQCYCIRHSFESDIVLASTVMDMYAKCGSIVDAKKVFDSTVEKDLILWNTLLAAYAESGLSGEALRLFYGMQLEGVPPNVITWNLIILSLLRNGQVDEAKDMFLQMQSSGIIPNLISWTTMMNGMVQNGCSEEAILFLRKMQESGLRPNAFSITVALSACAHLASLHIGRTIHGYIIRNLQHSSLVSIETSLVDMYAKCGDINKAEKVFGSKLYSELPLSNAMISAYALYGNLKEAIALYRSLEGVGLKPDNITITNVLSACNHAGDINQAIEIFTDIVSKRSMKPCLEHYGLMVDLLASAGETEKALRLIEEMPFKPDARMIQSLVASCNKQRKTELVDYLSRKLLESEPENSGNYVTISNAYAVEGSWDEVVKMREMMKAKGLKKKPGCSWIQITGEEGVHVFVANDKTHTRINEIQMMLALLLYDMGTGSK

SEQ ID NO: 4 - protein, 809 aa, Arabidopsis thaliana
MSSQLVQFSTVPQIPNPPSRHRHFLSERNYIPANVYEHPAALLLERCSSLKELRQILPLVFKNGLYQEHFFQTKLVSLFCRYGSVDEAARVFEPIDSKLNVLYHTMLKGFAKVSDLDKALQFFVRMRYDDVEPVVYNFTYLLKVCGDEAELRVGKEIHGLLVKSGFSLDLFAMTGLENMYAKCRQVNEARKVFDRMPERDLVSWNTIVAGYSQNGMARMALEMVKSMCEENLKPSFITIVSVLPAVSALRLISVGKEIHGYAMRSGFDSLVNISTALVDMYAKCGSLETARQLFDGMLERNVVSWNSMIDAYVQNENPKEAMLIFQKMLDEGVKPTDVSVMGALHACADLGDLERGRFIHKLSVELGLDRNVSVVNSLISMYCKCKEVDTAASMFGKLQSRTLVSWNAMILGFAQNGRPIDALNYFSQMRSRTVKPDTFTYVSVITAIAELSITHHAKWIHGVVMRSCLDKNVFVTTALVDMYAKCGAIMIARLIFDMMSERHVTTWNAMIDGYGTHGFGKAALELFEEMQKGTIKPNGVTFLSVISACSHSGLVEAGLKCFYMMKENYSIELSMDHYGAMVDLLGRAGRLNEAWDFIMQMPVKPAVNVYGAMLGACQIHKNVNFAEKAAERLFELNPDDGGYHVLLANIYRAASMWEKVGQVRVSMLRQGLRKTPGCSMVEIKNEVHSFFSGSTAHPDSKKIYAFLEKLICHIKEAGYVPDTNLVLGVENDVKEQLLSTHSEKLAISFGLLNTTAGTTIHVRKNLRVCADCHNATKYISLVTGREIVVRDMQRFHHFKNGACSCGDYW

SEQ ID NO: 5 - protein, 638 aa, Arabidopsis thaliana
MVVRSIIVSPPTTITYYHPMSIGLLVHPLSPHIPPASSPSASTAGNHHQRIFSLAETCSDMSQLKQLHAFTLRTTYPEEPATLFLYGKILQLSSSFSDVNYAFRVFDSIENHSSFMWNTLIRACAHDVSRKEEAFMLYRKMLERGESSPDKHTFPFVLKACAYIFGFSEGKQVHCQIVKHGFGGDVYVNNGLIHLYGSCGCLDLARKVFDEMPERSLVSWNSMIDALVRFGEYDSALQLFREMQRSFEPDGYTMQSVLSACAGLGSLSLGTWAHAFLLRKCDVDVAMDVLVKNSLIEMYCKCGSLRMAEQVFQGMQKRDLASWNAMILGFATHGRAEEAMNFFDRMVDKRENVRPNSVTFVGLLIACNHRGFVNKGRQYFDMMVRDYCIEPALEHYGCIVDLIARAGYITEAIDMVMSMPMKPDAVIWRSLLDACCKKGASVELSEEIARNIIGTKEDNESSNGNCSGAYVLLSRVYASASRWNDVGIVRKLMSEHGIRKEPGCSSIEINGISHEFFAGDTSHPQTKQIYQQLKVIDDRLRSIGYLPDRSQAPLVDATNDGSKEYSLRLHSERLAIAFGLINLPPQTPIRIFKNLRVCNDCHEVTKLISKVFNTEIIVRDRVRFHHFKDGSCSCLDYW

SEQ ID NO: 6 - protein, 613 aa, Arabidopsis thaliana
MLVFKSTMECSISSTIHVLGSCKTSDDVNQIHGRLIKTGIIKNSNLTTRIVLAFASSRRPYLADFARCVFHEYHVCSFSFGEVEDPFLWNAVIKSHSHGKDPRQALLLLCLMLENGVSVDKFSLSLVLKACSRLGFVKGGMQIHGFLKKTGLWSDLFLQNCLIGLYLKCGCLGLSRQMFDRMPKRDSVSYNSMIDGYVKCGLIVSARELFDLMPMEMKNLISWNSMISGYAQTSDGVDIASKLFADMPEKDLISWNSMIDGYVKHGRIEDAKGLFDVMPRRDVVTWATMIDGYAKLGFVHHAKTLFDQMPHRDVVAYNSMMAGYVQNKYHMEALEIFSDMEKESHLLPDDTTLVIVLPAIAQLGRLSKAIDMHLYIVEKQFYLGGKLGVALIDMYSKCGSIQHAMLVFEGIENKSIDHWNAMIGGLAIHGLGESAFDMLLQIERLSLKPDDITFVGVLNACSHSGLVKEGLLCFELMRRKHKIEPRLQHYGCMVDILSRSGSIELAKNLIEEMPVEPNDVIWRTFLTACSHHKEFETGELVAKHLILQAGYNPSSYVLLSNMYASFGMWKDVRRVRTMMKERKIEKIPGCSWIELDGRVHEFFVDSIEVSSTL

SEQ ID NO: 7 - protein, 684 aa, Arabidopsis thaliana
MSLLSADALGLLLKNAISASSMRLGRVVHARIVKTLDSPPPPFLANYLINMYSKLDHPESARLVLRLTPARNVVSWTSLISGLAQNGHFSTALVEFFEMRREGVVPNDFTFPCAFKAVASLRLPVTGKQIHALAVKCGRILDVFVGCSAFDMYCKTRLRDDARKLFDEIPERNLETWNAFISNSVTDGRPREAIEAFIEFRRIDGHPNSITFCAFLNACSDWLHLNLGMQLHGLVLRSGFDTDVSVCNGLIDFYGKCKQIRSSEIIFTEMGTKNAVSWCSLVAAYVQNHEDEKASVLYLRSRKDIVETSDFMISSVLSACAGMAGLELGRSIHAHAVKACVERTIFVGSALVDMYGKCGCIEDSEQAFDEMPEKNLVTRNSLIGGYAHQGQVDMALALFEEMAPRGCGPTPNYMTFVSLLSACSRAGAVENGMKIFDSMRSTYGIEPGAEHYSCIVDMLGRAGMVERAYEFIKKMPIQPTISVWGALQNACRMHGKPQLGLLAAENLFKLDPKDSGNHVLLSNTFAAAGRWAEANTVREELKGVGIKKGAGYSWITVKNQVHAFQAKDRSHILNKEIQTTLAKLRNEMEAAGYKPDLKLSLYDLEEEEKAAEVSHHSEKLALAFGLLSLPLSVPIRITKNLRICGDCHSFFKFVSGSVKREIIVRDNNRFHRFKDGICSCKDYW

SEQ ID NO: 8 - protein, 646 aa, Arabidopsis thaliana
MNPTQTLFSPGGNSPASSPASHPSSLFPQINNCRTIRDLSQIHAVFIKSGQMRDTLAAAEILRFCATSDLHHRDLDYAHKIFNQMPQRNCFSWNTIIRGFSESDEDKALIAITLFYEMMSDEFVEPNRFTFPSVLKACAKTGKIQEGKQIHGLALKYGFGGDEFVMSNLVRMYVMCGFMKDARVLFYKNIIEKDMVVMTDRRKRDGEIVLWNVMIDGYMRLGDCKAARMLFDKMRQRSVVSWNTMISGYSLNGFFKDAVEVFREMKKGDIRPNYVTLVSVLPAISRLGSLELGEWLHLYAEDSGIRIDDVLGSALIDMYSKCGIIEKAIHVFERLPRENVITWSAMINGFAIHGQAGDAIDCFCKMRQAGVRPSDVAYINLLTACSHGGLVEEGRRYFSQMVSVDGLEPRIEHYGCMVDLLGRSGLLDEAEEFILNMPIKPDDVIWKALLGACRMQGNVEMGKRVANILMDMVPHDSGAYVALSNMYASQGNWSEVSEMRLRMKEKDIRKDPGCSLIDIDGVLHEFVVEDDSHPKAKEINSMLVEISDKLRLAGYRPITTQVLLNLEEEDKENVLHYHSEKIATAFGLISTSPGKPIRIVKNLRICEDCHSSIKLISKVYKRKITVRDRKRFHHFQDGSCSCMDYW

SEQ ID NO: 9 - protein, 588 aa, Arabidopsis thaliana
MALNSSAFFVPCHNYNQICDLLLSSARTRSTIKGLQLHGYVVKSGLSLIPLVANNLINFYSKSQLPFDSRRAFEDSPQKSSTTWSSIISCFAQNELPWMSLEFLKKMMAGNLRPDDHVLPSATKSCAILSRCDIGRSVHCLSMKTGYDADVFVGSSLVDMYAKCGEIVYARKMFDEMPQRNVVTWSGMMYGYAQMGENEEALWLFKEALFENLAVNDYSFSSVISVCANSTLLELGRQIHGLSIKSSFDSSSFVGSSLVSLYSKCGVPEGAYQVFNEVPVKNLGIWNAMLKAYAQHSHTQKVIELFKRMKLSGMKPNFITFLNVLNACSHAGLVDEGRYYFDQMKESRIEPTDKHYASLVDMLGRAGRLQEALEVITNMPIDPTESVWGALLTSCTVHKNTELAAFAADKVFELGPVSSGMHISLSNAYAADGRFEDAAKARKLLRDRGEKKETGLSWVEERNKVHTFAAGERRHEKSKEIYEKLAELGEEMEKAGYIADTSYVLREVDGDEKNQTIRYHSERLAIAFGLITFPADRPIRVMKNLRVCGDCHNAIKFMSVCTRRVIIVRDNNRFHRFEDGKCSCNDYW

SEQ ID NO: 10 - protein, 659 aa, Arabidopsis thaliana
MKVRSKKALFCSVSRLLHTERHTERQNLTTLFNRYVDKTDVFSWNSVIADLARSGDSAEALLAFSSMRKLSLYPTRSSFPCAIKACSSLFDIFSGKQTHQQAFVFGYQSDIFVSSALIVMYSTCGKLEDARKVFDEIPKRNIVSWTSMIRGYDLNGNALDAVSLFKDLLVDENDDDDAMFLDSMGLVSVISACSRVPAKGLTESIHSFVIKRGFDRGVSVGNTLLDAYAKGGEGGVAVARKIFDQIVDKDRVSYNSIMSVYAQSGMSNEAFEVFRRLVKNKVVTFNAITLSTVLLAVSHSGALRIGKCIHDQVIRMGLEDDVIVGTSIIDMYCKCGRVETARKAFDRMKNKNVRSWTAMIAGYGMHGHAAKALELFPAMIDSGVRPNYITFVSVLAACSHAGLHVEGWRWFNAMKGRFGVEPGLEHYGCMVDLLGRAGFLQKAYDLIQRMKMKPDSIIWSSLLAACRIHKNVELAEISVARLFELDSSNCGYYMLLSHIYADAGRWKDVERVRMIMKNRGLVKPPGFSLLELNGEVHVFLIGDEEHPQREKIYEFLAELNRKLLEAGYVSNTSSVCHDVDEEEKEMTLRVHSEKLAIAFGIMNTVPGSTVNVVKNLRVCSDCHNVIKLISKIVDREFVVRDAKRFHHFKDGGCSCGDYW

SEQ ID NO: 11 - protein, 685 aa, Arabidopsis thaliana
MIKLIRFFRSRRCWVISLQARCFSAPSRTHFDFSGESSDTERALVSALGSCASSNDVTCGRQIHCRVLKSGLDSNGYICNSVLNMYAKCRLLADAESVFRDHAKLDSASFNIMVDGYVRSRRLWDALKLFDVMPERSCVSYTTLIKGYAQNNQWSEAMELFREMRNLGIMLNEVTLATVISACSHLGGIWDCRMLQSLAIKLKLEGRVFVSTNLLHMYCLCLCLKDARKLFDEMPERNLVTWNVMLNGYSKAGLIEQAEELFDQITEKDIVSWGTMIDGCLRKNQLDEALVYYTEMLRCGMKPSEVMMVDLLSASARSVGSSKGLQLHGTIVKRGFDCYDFLQATIIHFYAVSNDIKLALQQFEASVKDHIASRNALIAGFVKNGMVEQAREVFDQTHDKDIFSWNAMISGYAQSLSPQLALHLFREMISSSQVKPDAITMVSVFSAISSLGSLEEGKRAHDYLNFSTIPPNDNLTAAIIDMYAKCGSIETALNIFHQTKNISSSTISPWNAIICGSATHGHAKLALDLYSDLQSLPIKPNSITFVGVLSACCHAGLVELGKTYFESMKSDHGIEPDIKHYGCMVDLLGKAGRLEEAKEMIKKMPVKADVMIWGMLLSASRTHGNVEIAELAATELAAIDPSHGGCKVMLSNVYADAGRWEDVALVREEMRTRDVEWSRAFSGVV

SEQ ID NO: 12 - protein, 565 aa, Arabidopsis thaliana
MMKKHYKPILSQLENCRSLVELNQLHGLMIKSSVIRNVIPLSRLIDFCTTCPETMNLSYARSVFESIDCPSVYIWNSMIRGYSNSPNPDKALIFYQEMLRKGYSPDYFTFPYVLKACSGLRDIQFGSCVHGFVVKTGFEVNMYVSTCLLHMYMCCGEVNYGLRVFEDIPQWNVVAWGSLISGFVNNNRFSDAIEAFREMQSNGVKANETIMVDLLVACGRCKDIVTGKWFHGFLQGLGFDPYFQSKVGFNVILATSLIDMYAKCGDLRTARYLFDGMPERTLVSWNSIITGYSQNGDAEEALCMFLDMLDLGIAPDKVTFLSVIRASMIQGCSQLGQSIHAYVSKTGFVKDAAIVCALVNMYAKTGDAESAKKAFEDLEKKDTIAWTVVIIGLASHGHGNEALSIFQRMQEKGNATPDGITYLGVLYACSHIGLVEEGQRYFAEMRDLHGLEPTVEHYGCMVDILSRAGRFEEAERLVKTMPVKPNVNIWGALLNGCDIHENLELTDRIRSMVAEPEELGSGIYVLLSNIYAKAGRWADVKLIRESMKSKRVDKVLGHSSVETMF

SEQ ID NO: 13 - protein, 472 aa, Arabidopsis thaliana
MSSVFPGPRFLSLLQQNSKTLIQAKQIHAQLVINGCHDNSLFGKLIGHYCSKPSTESSSKLAHLLVFPRFGHPDKFLFNTLLKCSKPEDSIRIFANYASKSSLLYLNERTFVFVLGACARSASSSALRVGRIVHGMVKKLGFLYESELIGTTLLHFYAKNGDLRYARKVFDEMPERTSVTWNAMIGGYCSHKDKGNHNARKAMVLFRRFSCCGSGVRPTDTTMVCVLSAISQTGLLEIGSLVHGYIEKLGFTPEVDVFIGTALVDMYSKCGCLNNAFSVFELMKVKNVFTWTSMATGLALNGRGNETPNLLNRMAESGIKPNEITFTSLLSAYRHIGLVEEGIELFKSMKTRFGVTPVIEHYGCIVDLLGKAGRIQEAYQFILAMPIKPDAILLRSLCNACSIYGETVMGEEIGKALLEIEREDEKLSGSECEDYVALSNVLAHKGKWVEVEKLRKEMKERRIKTRPGYSFV

SEQ ID NO: 14 - protein, 534 aa, Arabidopsis thaliana
MAFHGIREVENYFIPFLQRVKSRNEWKKINASIIIHGLSQSSFMVTKMVDFCDKIEDMDYATRLFNQVSNPNVFLYNSIIRAYTHNSLYCDVIRIYKQLLRKSFELPDRFTFPFMFKSCASLGSCYLGKQVHGHLCKFGPRFHVVTENALIDMYMKFDDLVDAHKVFDEMYERDVISWNSLLSGYARLGQMKKAKGLFHLMLDKTIVSWTAMISGYTGIGCYVEAMDFFREMQLAGIEPDEISLISVLPSCAQLGSLELGKWIHLYAERRGFLKQTGVCNALIEMYSKCGVISQAIQLFGQMEGKDVISWSTMISGYAYHGNAHGAIETFNEMQRAKVKPNGITFLGLLSACSHVGMWQEGLRYFDMMRQDYQIEPKIEHYGCLIDVLARAGKLERAVEITKTMPMKPDSKIWGSLLSSCRTPGNLDVALVAMDHLVELEPEDMGNYVLLANIYADLGKWEDVSRLRKMIRNENMKKTPGGSLIEVNNIVQEFVSGDNSKPFWTEISIVLQLFTSHQDQDVITNNNALAFIGIV

SEQ ID NO: 15 - protein, 694 aa, Arabidopsis thaliana
MSEASCLASPLLYTNSGIHSDSFYASLIDSATHKAQLKQIHARLLVLGLQFSGFLITKLIHASSSFGDITFARQVFDDLPRPQIFPWNAIIRGYSRNNHFQDALLMYSNMQLARVSPDSFTFPHLLKACSGLSHLQMGRFVHAQVFRLGFDADVFVQNGLIALYAKCRRLGSARTVFEGLPLPERTIVSWTAIVSAYAQNGEPMEALEIFSQMRKMDVKPDWVALVSVLNAFTCLQDLKQGRSIHASVVKMGLEIEPDLLISLNTMYAKCGQVATAKILFDKMKSPNLILWNAMISGYAKNGYAREAIDMFHEMINKDVRPDTISITSAISACAQVGSLEQARSMYEYVGRSDYRDDVFISSALIDMFAKCGSVEGARLVFDRTLDRDVVVWSAMIVGYGLHGRAREAISLYRAMERGGVHPNDVTFLGLLMACNHSGMVREGWWFFNRMADHKINPQQQHYACVIDLLGRAGHLDQAYEVIKCMPVQPGVTVWGALLSACKKHRHVELGEYAAQQLFSIDPSNTGHYVQLSNLYAAARLWDRVAEVRVRMKEKGLNKDVGCSWVEVRGRLEAFRVGDKSHPRYEEIERQVEWIESRLKEGGFVANKDASLHDLNDEEAEETLCSHSERIAIAYGLISTPQGTPLRITKNLRACVNCHAATKLISKLVDREIVVRDTNRFHHFKDGVCSCGDYW

SEQ ID NO: 16 - protein, 656 aa, Arabidopsis thaliana
MIRSRSVLLIFRKVLYQSSCLKCLLCANSFSTSVSSSLGFRATNKELNQMIRSGYIAEARDIFEKLEARNTVTWNTMISGYVKRREMNQARKLFDVMPKRDVVTWNTMISGYVSCGGIRFLEEARKLFDEMPSRDSFSWNTMISGYAKNRRIGEALLLFEKMPERNAVSWSAMITGFCQNGEVDSAVVLFRKMPVKDSSPLCALVAGLIKNERLSEAAWVLGQYGSLVSGREDLVYAYNTLIVGYGQRGQVEAARCLFDQIPDLCGDDHGGEFRERFCKNVVSWNSMIKAYLKVGDVVSARLLFDQMKDRDTISWNTMIDGYVHVSRMEDAFALFSEMPNRDAHSWNMMVSGYASVGNVELARHYFEKTPEKHTVSWNSIIAAYEKNKDYKEAVDLFIRMNIEGEKPDPHTLTSLLSASTGLVNLRLGMQMHQIVVKTVIPDVPVHNALITMYSRCGEIMESRRIFDEMKLKREVITWNAMIGGYAFHGNASEALNLFGSMKSNGIYPSHITFVSVLNACAHAGLVDEAKAQFVSMMSVYKIEPQMEHYSSLVNVTSGQGQFEEAMYIITSMPFEPDKTVWGALLDACRIYNNVGLAHVAAEAMSRLEPESSTPYVLLYNMYADMGLWDEASQVRMNMESKRIKKERGSSWVDSST

SEQ ID NO: 17 - protein, 544 aa, Arabidopsis thaliana
MISSLAAITGGPSTFRRDPDSNTLRLSRRKTLISVLRSCKNIAHVPSIHAKIIRTFHDQDAFVVFELIRVCSTLDSVDYAYDVFSYVSNPNVYLYTAMIDGFVSSGRSADGVSLYHRMIHNSVLPDNYVITSVLKACDLKVCREIHAQVLKLGFGSSRSVGLKMMEIYGKSGELVNAKKMFDEMPDRDHVAATVMINCYSECGFIKEALELFQDVKIKDTVCWTAMIDGLVRNKEMNKALELFREMQMENVSANEFTAVCVLSACSDLGALELGRWVHSFVENQRMELSNFVGNALINMYSRCGDINEARRVFRVMRDKDVISYNTMISGLAMHGASVEAINEFRDMVNRGFRPNQVTLVALLNACSHGGLLDIGLEVFNSMKRVFNVEPQIEHYGCIVDLLGRVGRLEEAYRFIENIPIEPDHIMLGTLLSACKIHGNMELGEKIAKRLFESENPDSGTYVLLSNLYASSGKWKESTEIRESMRDSGIEKEPGCSTIEVDNQIHEFLVGDIAHPHKEAIYQRLQELNRILRFKENQIDIIMGF

SEQ ID NO: 18 - protein, 738 aa, Arabidopsis thaliana
MAIFSTAQPLSLPRHPNFSNPNQPTTNNERSRHISLIERCVSLRQLKQTHGHMIRTGTFSDPYSASKLFAMAALSSFASLEYARKVFDEIPKPNSFAWNTLIRAYASGPDPVLSIWAFLDMVSESQCYPNKYTFPFLIKAAAEVSSLSLGQSLHGMAVKSAVGSDVFVANSLIHCYFSCGDLDSACKVFTTIKEKDVVSWNSMINGFVQKGSPDKALELFKKMESEDVKASHVTMVGVLSACAKIRNLEFGRQVCSYIEENRVNVNLTLANAMLDMYTKCGSIEDAKRLFDAMEEKDNVTWTTMLDGYAISEDYEAAREVLNSMPQKDIVAWNALISAYEQNGKPNEALIVFHELQLQKNMKLNQITLVSTLSACAQVGALELGRWIHSYIKKHGIRMNFHVTSALIHMYSKCGDLEKSREVFNSVEKRDVFVWSAMIGGLAMHGCGNEAVDMFYKMQEANVKPNGVTFTNVFCACSHTGLVDEAESLFHQMESNYGIVPEEKHYACIVDVLGRSGYLEKAVKFIEAMPIPPSTSVWGALLGACKIHANLNLAEMACTRLLELEPRNDGAHVLLSNIYAKLGKWENVSELRKHMRVTGLKKEPGCSSIEIDGMIHEFLSGDNAHPMSEKVYGKLHEVMEKLKSNGYEPEISQVLQIIEEEEMKEQSLNLHSEKLAICYGLISTEAPKVIRVIKNLRVCGDCHSVAKLISQLYDREIIVRDRYRFHHFRNGQCSCNDFW

SEQ ID NO: 19 - protein, 741 aa, Arabidopsis thaliana
MMLSCSPLTVPSSSYPFHFLPSSSDPPYDSIRNHPSLSLLHNCKTLQSLRIIHAQMIKIGLHNTNYALSKLIEFCILSPHFEGLPYAISVFKTIQEPNLLIWNTMFRGHALSSDPVSALKLYVCMISLGLLPNSYTFPFVLKSCAKSKAFKEGQQIHGHVLKLGCDLDLYVHTSLISMYVQNGRLEDAHKVFDKSPHRDVVSYTALIKGYASRGYIENAQKLFDEIPVKDVVSWNAMISGYAETGNYKEALELFKDMMKTNVRPDESTMVTVVSACAQSGSIELGRQVHLWIDDHGFGSNLKIVNALIDLYSKCGELETACGLFERLPYKDVISWNTLIGGYTHMNLYKEALLLFQEMLRSGETPNDVTMLSILPACAHLGAIDIGRWIHVYIDKRLKGVTNASSLRTSLIDMYAKCGDIEAAHQVFNSILHKSLSSWNAMIFGFAMHGRADASFDLFSRMRKIGIQPDDITFVGLLSACSHSGMLDLGRHIFRTMTQDYKMTPKLEHYGCMIDLLGHSGLFKEAEEMINMMEMEPDGVIWCSLLKACKMHGNVELGESFAENLIKIEPENPGSYVLLSNIYASAGRWNEVAKTRALLNDKGMKKVPGCSSIEIDSVVHEFIIGDKFHPRNREIYGMLEEMEVLLEKAGFVPDTSEVLQEMEEEWKEGALRHHSEKLAIAFGLISTKPGTKLTIVKNLRVCRNCHEATKLISKIYKREIIARDRTRFHHFRDGVCSCNDYW

SEQ ID NO: 20 - protein, 890 aa, Arabidopsis thaliana
MSCPLAFTFSLPSIFPFPSQLLPFSRHKHPYLLRATPTSATEDVASAVSGAPSIFISQSRSPEWWIDLLRSKVRSNLLREAVLTYVDMIVLGIKPDNYAFPALLKAVADLQDMELGKQIHAHVYKFGYGVDSVTVANTLVNLYRKCGDFGAVYKVFDRISERNQVSWNSLISSLCSFEKWEMALEAFRCMLDENVEPSSFTLVSVVTACSNLPMPEGLMMGKQVHAYGLRKGELNSFIINTLVAMYGKLGKLASSKVLLGSFGGRDLVTWNTVLSSLCQNEQLLEALEYLREMVLEGVEPDEFTISSVLPACSHLEMLRTGKELHAYALKNGSLDENSFVGSALVDMYCNCKQVLSGRRVFDGMFDRKIGLWNAMIAGYSQNEHDKEALLLFIGMEESAGLLANSTTMAGVVPACVRSGAFSRKEAIHGFVVKRGLDRDRFVQNTLMDMYSRLGKIDIAMRIFGKMEDRDLVTWNTMITGYVFSEHHEDALLLLHKMQNLERKVSKGASRVSLKPNSITLMTILPSCAALSALAKGKEIHAYAIKNNLATDVAVGSALVDMYAKCGCLQMSRKVFDQIPQKNVITWNVIIMAYGMHGNGQEAIDLLRMMMVQGVKPNEVTFISVFAACSHSGMVDEGLRIFYVMKPDYGVEPSSDHYACVVDLLGRAGRIKEAYQLMNMMPRDFNKAGAWSSLLGASRIHNNLEIGEIAAQNLIQLEPNVASHYVLLANIYSSAGLWDKATEVRRNMKEQGVRKEPGCSWIEHGDEVHKFVAGDSSHPQSEKLSGYLETLWERMRKEGYVPDTSCVLHNVEEDEKEILLCGHSEKLAIAFGILNTSPGTIIRVAKNLRVCNDCHLATKFISKIVDREIILRDVRRFHRFKNGTCSCGDYW

SEQ ID NO: 21 - protein, 603 aa, Arabidopsis thaliana
MAISSASLISSFSHAETFTKHSKIDTVNTQNPILLISKCNSLRELMQIQAYAIKSHIEDVSFVAKLINFCTESPTESSMSYARHLFEAMSEPDIVIFNSMARGYSRFTNPLEVFSLFVEILEDGILPDNYTFPSLLKACAVAKALEEGRQLHCLSMKLGLDDNVYVCPTLINMYTECEDVDSARCVFDRIVEPCVVCYNAMITGYARRNRPNEALSLFREMQGKYLKPNEITLLSVLSSCALLGSLDLGKWIHKYAKKHSFCKYVKVNTALIDMFAKCGSLDDAVSIFEKMRYKDTQAWSAMIVAYANHGKAEKSMLMFERMRSENVQPDEITFLGLLNACSHTGRVEEGRKYFSQMVSKFGIVPSIKHYGSMVDLLSRAGNLEDAYEFIDKLPISPTPMLWRILLAACSSHNNLDLAEKVSERIFELDDSHGGDYVILSNLYARNKKWEYVDSLRKVMKDRKAVKVPGCSSIEVNNVVHEFFSGDGVKSATTKLHRALDEMVKELKLSGYVPDTSMVVHANMNDQEKEITLRYHSEKLAITFGLLNTPPGTTIRVVKNLRVCRDCHNAAKLISLIFGRKVVLRDVQRFHHFEDGKCSCGDFW

SEQ ID NO: 22 - protein, 960 aa, Arabidopsis thaliana
MEYAVTNMRLLSNMMYSASAISFPRVRLHCSIPTEPSCRRNPFRQSNQPVQVPSPKLACFDGVLTEAFQRLDVSENNSPVEAFAYVLELCGKRRAVSQGRQLHSRIFKTFPSFELDFLAGKLVFMYGKCGSLDDAEKVFDEMPDRTAFAWNTMIGAYVSNGEPASALALYWNMRVEGVPLGLSSFPALLKACAKLRDIRSGSELHSLLVKLGYHSTGFIVNALVSMYAKNDDLSAARRLFDGFQEKGDAVLWNSILSSYSTSGKSLETLELFREMHMTGPAPNSYTIVSALTACDGFSYAKLGKEIHASVLKSSTHSSELYVCNALIAMYTRCGKMPQAERILRQMNNADVVTWNSLIKGYVQNLMYKEALEFFSDMIAAGHKSDEVSMTSIIAASGRLSNLLAGMELHAYVIKHGWDSNLQVGNTLIDMYSKCNLTCYMGRAFLRMHDKDLISWTTVIAGYAQNDCHVEALELFRDVAKKRMEIDEMILGSILRASSVLKSMLIVKEIHCHILRKGLLDTVIQNELVDVYGKCRNMGYATRVFESIKGKDVVSWTSMISSSALNGNESEAVELFRRMVETGLSADSVALLCILSAAASLSALNKGREIHCYLLRKGFCLEGSIAVAVVDMYACCGDLQSAKAVFDRIERKGLLQYTSMINAYGMHGCGKAAVELFDKMRHENVSPDHISFLALLYACSHAGLLDEGRGFLKIMEHEYELEPWPEHYVCLVDMLGRANCVVEAFEFVKMMKTEPTAEVWCALLAACRSHSEKEIGEIAAQRLLELEPKNPGNLVLVSNVFAEQGRWNDVEKVRAKMKASGMEKHPGCSWIEMDGKVHKFTARDKSHPESKEIYEKLSEVTRKLEREVGYVADTKFVLHNVDEGEKVQMLHGHSERIAIAYGLLRTPDRACLRITKNLRVCRDCHTFCKLVSKLFRRDIVMRDANRFHHFESGLCSCGDSW

SEQ ID NO: 23 - protein, 895 aa, Arabidopsis thaliana
MNCLANESLNSLKISPFSTSRLLSSVTNFRNQLSFSSKDSSSSSAPFNPFRFFNDQSNSRLCNLRTTKILQAHLLRRYLLPFDVFLTKSLLSWYSNSGSMADAAKLFDTIPQPDVVSCNIMISGYKQHRLFEESLRFFSKMHFLGFEANEISYGSVISACSALQAPLFSELVCCHTIKMGYFFYEVVESALIDVFSKNLRFEDAYKVFRDSLSANVYCWNTIIAGALRNQNYGAVFDLFHEMCVGFQKPDSYTYSSVLAACASLEKLRFGKVVQARVIKCGAEDVFVCTAIVDLYAKCGHMAEAMEVFSRIPNPSVVSWTVMLSGYTKSNDAFSALEIFKEMRHSGVEINNCTVTSVISACGRPSMVCEASQVHAWVFKSGFYLDSSVAAALISMYSKSGDIDLSEQVFEDLDDIQRQNIVNVMITSFSQSKKPGKAIRLFTRMLQEGLRTDEFSVCSLLSVLDCLNLGKQVHGYTLKSGLVLDLTVGSSLFTLYSKCGSLEESYKLFQGIPFKDNACWASMISGFNEYGYLREAIGLFSEMLDDGTSPDESTLAAVLTVCSSHPSLPRGKEIHGYTLRAGIDKGMDLGSALVNMYSKCGSLKLARQVYDRLPELDPVSCSSLISGYSQHGLIQDGFLLFRDMVMSGFTMDSFAISSILKAAALSDESSLGAQVHAYITKIGLCTEPSVGSSLLTMYSKFGSIDDCCKAFSQINGPDLIAWTALIASYAQHGKANEALQVYNLMKEKGFKPDKVTFVGVLSACSHGGLVEESYFHLNSMVKDYGIEPENRHYVCMVDALGRSGRLREAESFINNMHIKPDALVWGTLLAACKIHGEVELGKVAAKKAIELEPSDAGAYISLSNILAEVGEWDEVEETRKLMKGTGVQKEPGWSSV

SEQ ID NO: 24 - protein, 681 aa, Arabidopsis thaliana
MNISKAKLLLLPPPLTPKLNRSLYSHSQRRTRSLPHHRDKPINWNSTHSFVLHNPLLSLLEKCKLLLHLKQIQAQMIINGLILDPFASSRLIAFCALSESRYLDYSVKILKGIENPNIFSWNVTIRGFSESENPKESFLLYKQMLRHGCCESRPDHFTYPVLFKVCADLRLSSLGHMILGHVLKLRLELVSHVHNASIHMFASCGDMENARKVFDESPVRDLVSWNCLINGYKKIGEAEKAIYVYKLMESEGVKPDDVTMIGLVSSCSMLGDLNRGKEFYEYVKENGLRMTIPLVNALMDMFSKCGDIHEARRIFDNLEKRTIVSWTTMISGYARCGLLDVSRKLFDDMEEKDVVLWNAMIGGSVQAKRGQDALALFQEMQTSNTKPDEITMIHCLSACSQLGALDVGIWIHRYIEKYSLSLNVALGTSLVDMYAKCGNISEALSVFHGIQTRNSLTYTAIIGGLALHGDASTAISYFNEMIDAGIAPDEITFIGLLSACCHGGMIQTGRDYFSQMKSRFNLNPQLKHYSIMVDLLGRAGLLEEADRLMESMPMEADAAVWGALLFGCRMHGNVELGEKAAKKLLELDPSDSGIYVLLDGMYGEANMWEDAKRARRMMNERGVEKIPGCSSIEVNGIVCEFIVRDKSRPESEKIYDRLHCLGRHMRSSLSVLFSEYEITNN

SEQ ID NO: 25 - protein, 842 aa, Arabidopsis thaliana
MAMLGNVLHLSPMVLATTTTTKPSLLNQSKCTKATPSSLKNCKTIDELKMFHRSLTKQGLDNDVSTITKLVARSCELGTRESLSFAKEVFENSESYGTCFMYNSLIRGYASSGLCNEAILLFLRMMNSGISPDKYTFPFGLSACAKSRAKGNGIQIHGLIVKMGYAKDLFVQNSLVHFYAECGELDSARKVFDEMSERNVVSWTSMICGYARRDFAKDAVDLFFRMVRDEEVTPNSVTMVCVISACAKLEDLETGEKVYAFIRNSGIEVNDLMVSALVDMYMKCNAIDVAKRLFDEYGASNLDLCNAMASNYVRQGLTREALGVFNLMMDSGVRPDRISMLSAISSCSQLRNILWGKSCHGYVLRNGFESWDNICNALIDMYMKCHRQDTAFRIFDRMSNKTVVTWNSIVAGYVENGEVDAAWETFETMPEKNIVSWNTIISGLVQGSLFEEAIEVFCSMQSQEGVNADGVTMMSIASACGHLGALDLAKWIYYYIEKNGIQLDVRLGTTLVDMFSRCGDPESAMSIFNSLTNRDVSAWTAAIGAMAMAGNAERAIELFDDMIEQGLKPDGVAFVGALTACSHGGLVQQGKEIFYSMLKLHGVSPEDVHYGCMVDLLGRAGLLEEAVQLIEDMPMEPNDVIWNSLLAACRVQGNVEMAAYAAEKIQVLAPERTGSYVLLSNVYASAGRWNDMAKVRLSMKEKGLRKPPGTSSIQIRGKTHEFTSGDESHPEMPNIEAMLDEVSQRASHLGHVPDLSNVLMDVDEKEKIFMLSRHSEKLAMAYGLISSNKGTTIRIVKNLRVCSDCHSFAKFASKVYNREIILRDNNRFHYIRQGKCSCGDFW

SEQ ID NO: 26 - protein, 859 aa, Physcomitrella patens
MLHQGAGRARGGLPSLLLGRRFDLWASFPWSFSSTSDDPSSRQSEENSQTIDELWEYFAGPSQWWDNRIHKRNPRSPDLKHKVTGKALWIDGCFTPEWVKFQPVAQVGLQSYATCTTKCTEGGAQGKRQPKGNDGKLATACESARVLGRIAQGGINMHVQTANTLSEAIVVLMNRLQRGLITDSFMYVEVLKRCLKQKDLMAAKQVHDCIIKSRMEQNAHVMNNLLHVYIECGRLQEARCVFDALVKKSGASWNAMIAGYVEHKHAEDAMRLFREMCHEGVQPNAGTYMIILKACASLSALKWGKEVHACIRHGGLESDVRVGTALLRMYGKCGSINEARRIFDNLMNHDIISWTVMIGAYAQSGNGKEAYRLMLQMEQEGFKPNAITYVSILNACASEGALKWVKRVHRHALDAGLELDVRVGTALVQMYAKSGSIDDARVVFDRMKVRDVVSWNVMIGAFAEHGRGHEAYDLFLQMQTEGCKPDAIMFLSILNACASAGALEWVKKIHRHALDSGLEVDVRVGTALVHMYSKSGSIDDARVVFDRMKVRNVVSWNAMISGLAQHGLGQDALEVFRRMTAHGVKPDRVTFVAVLSACSHAGLVDEGRSQYLAMTQVYGIEPDVSHCNCMVDLLGRAGRLMEAKLFIDNMAVDPDEATWGALLGSCRTYGNVELGELVAKERLKLDPKNAATYVLLSNIYAEAGKWDMVSWVRTMMRERGIRKEPGRSWIEVDNKIHDFLVADSSHPECKEINESKDKVIEKIKAEGYIPDTRLVLKNKNMKDKELDICSHSEKLAIVYGLMHTPPGNPIRVFKNLRVCTDCHGATKLISKVEGREIIVRDANRFHHFKDGVCSCGDYW

SEQ ID NO: 27 - protein, 833 aa, Physcomitrella patens
MRVSTRIAANIAVVRRRWFGSLQLPVPSARFRSTFTRRVGANDVLQRLGEGGNHIDSRTYVKLFQRCTELRDAALGKQVRDHIIQGGRQLNIYELNTLIKLYSICGNVTEARQIFDSVENKTVVTWNALIAGYAQVGHVKEAFALFRQMVDEGLEPSIITFLSVLDACSSPAGLNWGKEVHAQVVTAGFVSDFRIGTALVSMYVKGGSMDDARQVFDGLHIRDVSTFNVMVGGYAKSGDWEKAFELFYRMQQVGLKPNKISFLSILDGCWTPEALAWGKAVHAQCMNAGLVDDIRVATSLIRMYTTCGSIEGARRVFDNMKVRDVVSWTVMIEGYAENGNIEDAFGLFATMQEEGIQPDRITYMHIMNACAISANLNHAREIHSQVDIAGFGTDLLVSTALVHMYAKCGAIKDARQVFDAMPRRDVVSWSAMIGAYVENGYGTEAFETFHLMKRSNIEPDGVTYINLLNACGHLGALDVGMEIYTQAIKADLVSHVPLGNALIIMNAKHGSVERARYIFDTMVRRDVITWNAMIGGYSLHGNAREALYLFDRMLKERFRPNSVTFVGVLSACSRAGFVDEGRRFFTYLLEGRGIVPTVKLYGCMVDLLGRAGELDEAELLIKSMPVKPTSSIWSSLLVACRIHGNLDVAERAAERCLMIDPYDGAVYVQLSHMYAAAGMWENVAKVRKVMESRGIRKEQGCTWIEVAGKVHTFVVEDRSHPLVGEIYAELARLMNAIKREGYIPITQNVLHDVGEQQKEEAISYHSEKLAIAYGVLSLPSGTPIRIYKNLRVCSDCHSASKFISKVTGREIIARDASRFHHFKDGVCSCGDYW

SEQ ID NO: 28 - protein, 1204 aa, Physcomitrella patens
MYRCLWRSVIQTHKGSLGRVAGVREFSARPWPVEQNRSSIGAAGGESSNLVPVKVMRNERHCGPDREDVSNTHQPRPTETDRATYVALLQNCTRKRLLMRNERHCGPDREDVSNTHQPRPTETERATYVALLQNCTRKRLLPEAKRIHAQMVEAWVGPDIFLSNLLINMYVKCRSVLDAHQVFKEMPRRDVISWNSLISCYAQQGFKKKAFQLFEEMQNAGFIPNKITYISILTACYSPAELENGKKIHSQIIKAGYQRDPRVQNSLLSMYGKCGDLPRARQVFAGISPRDVVSYNTMLGLYAQKAYVKECLGLFGQMSSEGISPDKVTYINLLDAFTTPSMLDEGKRIHKLTVEEGLNSDIRVGTALVTMCVRCGDVDSAKQAFKGTADRDVVVYNALIAALAQHGHNVEAFEQYYRMRSDGVALNRTTYLSILNACSTSKALEAGKLIHSHISEDGHSSDVQIGNALISMYARCGDLPKARELFYTMPKRDLISWNAIIAGYARREDRGEAMRLYKQMQSEGVKPGRVTFLHLLSACANSSAYADGKMIHEDILRSGIKSNGHLANALMNMYRRCGSLMEAQNVFEGTQARDVISWNSMIAGHAQHGSYETAYKLFQEMQNEELEPDNITFASVLSGCKNPEALELGKQIHGRITESGLQLDVNLGNALINMYIRCGSLQDARNVFHSLQHRDVMSWTAMIGGCADQGEDMKAIELFWQMQNEGFRPVKSTFSSILKVCTSSACLDEGKKVIAYILNSGYELDTGVGNALISAYSKSGSMTDAREVFDKMPSRDIVSWNKIIAGYAQNGLGQTAVEFAYQMQEQDVVPNKFSFVSLLNACSSFSALEEGKRVHAEIVKRKLQGDVRVGAALISMYAKCGSQGEAQEVFDNIIEKNVVTWNAMINAYAQHGLASKALGFFNCMEKEGIKPDGSTFTSILSACNHAGLVLEGYQIFSSMESEYGVLPTIEHYGCLVGLLGRARRFQEAETLINQMPFPPDAAVWETLLGACRIHGNIALAEHAANNALKLNARNPAVYILLSNVYAAAGRWDDVAKIRRVMEGRGIRKEPGRSWIEVDNIIHEFIAADRSHPETAEIYAELKRLSVEMEEAGYFPDTQHVLHDLGKAHQETSLCTHSERLAIAYGLIKTPPGTPIRIFKNLRICGDCHTASKFISKLVGREIIARDSNRFHSFKNGKCSCEDYW

SEQ ID NO: 29 - protein, 1042 aa, Physcomitrella patens
MSLPWGLDFTTVSTAKQTQAGFSVLKKEKHSLRDDLILATSRQNDAGHKIDLVGDSARNFLVKQIARDSDTLVRADLKKECSRAYGKPSLLVEAHRSSSMHSQSRVQLCKWWFNTSGFRYSNGKPRVNKLYFHTYKDEKIMIEKDGAVDVVQYLQQQGAQVNSSDYMKMLKRCIEVKDLVAGRQVHQHIIQHRTVPDQYTVNALINMYIQCGSIEEARQVWKKLSYMERTVHSWNAMVVGYIQYGYIEKALKLLRQMQQHGLAPDRTTIMSFLSSCKSPGALEWGREIHFQAMQAGLLFDVKVANCILNMYAKCGSIEEAREVFDKMEKKSVVSWTITIGGYADCGRSETAFEIFQKMEQEGVVPNRITYISVLNAFSSPAALKWGKAVHSRILNAGHESDTAVGTALVKMYAKCGSYKDCRQVFEKLVNRDLIAWNTMIGGLAEGGYWEEASEVYNQMQREGVMPNKITYVILLNACVNSAALHWGKEIHSRVAKAGFTSDIGVQNALISMYSRCGSIKDARLVFDKMVRKDVISWTAMIGGLAKSGFGAEALTVYQEMQQAGVEPNRVTYTSILNACSSPAALEWGRRIHQQVVEAGLATDAHVGNTLVNMYSMCGSVKDARQVFDRMIQRDIVAYNAMIGGYAAHNLGKEALKLFDRLQEEGLKPDKVTYINMLNACANSGSLEWAREIHTLVRKGGFFSDTSVGNALVSTYAKCGSFSDASIVFEKMTKRNVISWNAIIGGSAQHGRGQDALQLFERMKMEGVKPDIVTFVSLLSACSHAGLLEEGRRYFCSMSQDFAIIPTIEHYGCMVDLLGRAGQLDEAEALIKTMPFQANTRIWGALLGACRIHGNVPVAERAAESSLKLDLDNAVVYVALSHMYAAAGMWDSAAKLRKLMEQRGVTKEPGRSWIQVGDKLHYFVAEDRSHPQSEKIYAELDRLTHAMKMKGYVPDTRSVMHDVDEGEKENAVCHHSERLAIAYGLISTPPGTRIHIFKNLRVCPDCHTATKFISKIVDREIIARDVNRFHHFKDGVCSCGDYW

SEQ ID NO: 30 - protein, 804 aa, Physcomitrella patens
MIPTGKDGWYAPADVLQYLHRKGPQVDSYDYVKLLQSCVKAKDLAVGKQVHEHILRCGVKPNVYITNTLLKLYAHCGSVNEARQLFDKFSNKSVVSWNVMISGYAHRGLAQEAFNLFTLMQQERLEPDKFTFVSILSACSSPAVLNWGREIHVRVMEAGLANDTTVGNALISMYAKCGSVRDARRVFDAMASRDEVSWTTLTGAYAESGYGEESLKTYHAMLQERVRPSRITYMNVLSACGSLAALEKGKQIHAHIVESEYHSDVRVSTALTKMYMKCGAFKDAREVFECLSYRDVIAWNTMIRGFVDSGQLEEAHGTFHRMLEEGVAPDRATYTTVLSACARPGGLARGKEIHARAAKDGLVSDVRFGNALINMYSKAGSMKDARQVFDRMPKRDVVSWTTLLGRYADCDQVVESFTTFKQMLQQGVKANKITYMCVLKACSNPVALKWGKEIHAEVVKAGLLADLAVTNALMSMYFKCGSVEDAIRVFEGMSMRDVVTWNTLIGGLGQNGRGLEALQRYEVMKSEGMRPNAATFVNVLSACRVCNLVEEGRRQFAFMSKDYGIVPTEKHYACMVDILARAGHLREAEDVILTIPLKPSAAMWGALLAACRIHCNVEIGERAAEHCLKLEPQNAGLYVSLSAIYAAAGMWRDVAKLRKFMKERGVKKEPGRSWIEIAGEVHSFVARDQSHPRTQEIYAELETLKKQMKSLGYVPDTRFVMHDLDDEGKERAVCHHSEKLAIAYGLISTPPGTPIRISKNLRVCTDCHTATKFISKITKREIIARDAHRFHHFKNGECSCGDYW

SEQ ID NO: 31 - protein, 890 aa, Physcomitrella patens
MLSRRFGLRRWKQVLQNYHVGAMTSIVYNDGFASTGKELDGPTSVSGGEVWRLCKAGRLREAIQLLGIIKQRGLLVNSNTYGCVIEHCAKARRFEDGKMVHKQLDELGVEIDIYLGNSLINFYSKFEDVASAEQVFRRMTLRDVVTWSSMIAAYAGNNHPAKAFDTFERMTDANIEPNRITFLSILKACNNYSILEKGRKIHTIVKAMGMETDVAVATALITMYSKCGEISVACEVFHKMTERNVVSWTAIIQANAQHRKLNEAFELYEQMLQAGISPNAVTFVSLLNSCNTPEALNRGRRIHSHISERGLETDMIVANALITMYCKCNSVQEAREIFDRMSKRDVISWSAMIAGYAQSGYKDKESIDEVFQLLERMRREGVFPNKVTFMSILRACTAHGALEQGRQIHAELSKVGFELDRSLQTAIFNMYAKCGSIYEAEQVFSKMANKNVVAWTSFLSMYIKCGDLSSAEKVFSEMPTRNVVSWNLMIAGYAQNGDIVKVFELLSSMKAEGFQPDRVTVITILEACGALAGLERGKLVHAEAVKLGLESDTVVATSLIGMYSKCGQVAEARTVFDKMSNRDTVAWNAMLAGYGQHGDGLEAVDLFKRMLKERVSPNEITLTAVISACSRAGLVQEGREIFRMMQEDFKMTPRKQHYGCMVDLLGRAGRLQEAEEFIQSMPCEPDISVWHALLGACKSHNNVQLAERAAHHILELEPSYASVYITLSNIYAQAGRWDDSTKVRRVMDDRGLKKDRGESSIEIDGRIHTFVAEDCAHPEIDAIHAELETLTKEMKEAGYTPDMRFVLHDVDDVQKEKALCHHSEKLAIAYGLLKTPSGTPIRIMKNLRVCGDCHTATKFISKIRKREIVARDANRFHYFNNGTCSCGDFW

SEQ ID NO: 32 - RNA, 31 nt, Physcomitrella patens
cuauagguauuggaaacguauuuaguucuuc

SEQ ID NO: 33 - RNA, 31 nt, Physcomitrella patens
cuauuucaaugguugguaaguagagauguuc

SEQ ID NO: 34 - RNA, 31 nt, Physcomitrella patens
guagagauguuuccacaggugcuccuuuuuc

SEQ ID NO: 35 - RNA, 31 nt, Physcomitrella patens
aucccgauccugaggucuauauucuaauuuc

SEQ ID NO: 36 - RNA, 31 nt, Physcomitrella patens
acaauuacuaucaaagcuauuggacaucaac

SEQ ID NO: 37 - RNA, 31 nt, Physcomitrella patens
cacuuuggcuuugaagcagcugcuugguacc

SEQ ID NO: 38 - RNA, 31 nt, Physcomitrella patens
uuauuauauuugauuuggaagucaccuuuuc

SEQ ID NO: 39 - RNA, 31 nt, Physcomitrella patens
auuuuuauauagguauagacgguaucucuuc

SEQ ID NO: 40 - RNA, 31 nt, Physcomitrella patens
caaacaguagacuuuucgacuauuuuugcuc

SEQ ID NO: 41 - RNA, 31 nt, Physcomitrella patens
ggaaaaucugcacaaauaggauugcauacuc

SEQ ID NO: 42 - RNA, 31 nt, Physcomitrella patens
cuaaaacaaauauuuuaauaauaaaaaaauc

SEQ ID NO: 43 - RNA, 31 nt, Physcomitrella patens
aaaacaaauauuuuaauaauaaaaaaaucac

SEQ ID NO: 44 - RNA, 31 nt, Physcomitrella patens
aucaaauacguuaugaauauuuuuuaaaguc

SEQ ID NO: 45 - RNA, 31 nt, Arabidopsis thaliana
aaaugaguaguucagaaagaaucgagcuuuc

SEQ ID NO: 46 - RNA, 31 nt, Arabidopsis thaliana
uuuuuuuuaucgauauucuuguuuacuacuc

SEQ ID NO: 47 - RNA, 31 nt, Arabidopsis thaliana
gauuuaauaccgauauuuuagcaacaaaucc

SEQ ID NO: 48 - RNA, 31 nt, Arabidopsis thaliana
guuuuuaugucagcaacagaagcccaagcuc

SEQ ID NO: 49 - RNA, 31 nt, Arabidopsis thaliana
ccaagauuuuucuuguucuuauauaauucuc

SEQ ID NO: 50 - RNA, 31 nt, Arabidopsis thaliana
ugauuguaugugugauagcaucuacuauacc

SEQ ID NO: 51 - RNA, 31 nt, Arabidopsis thaliana
ccuccacuagcagguuuuuuuggaaaacucc

SEQ ID NO: 52 - RNA, 31 nt, Arabidopsis thaliana
cucgaauuuucgauauuccuuuuuauuucuc

SEQ ID NO: 53 - RNA, 31 nt, Arabidopsis thaliana
cuguuacuucgaaaguagcugcuucagcuuc

SEQ ID NO: 54 - RNA, 31 nt, Arabidopsis thaliana
uucuuucuguuacuucgaaaguagcugcuuc

SEQ ID NO: 55 - RNA, 31 nt, Arabidopsis thaliana
gaauuggguucaagcuuucccuagccccuuc

SEQ ID NO: 56 - RNA, 31 nt, Arabidopsis thaliana
auggguggggcaagcucuucuauucugguuc

SEQ ID NO: 57 - RNA, 31 nt, Arabidopsis thaliana
cuaacgauuuaauaacuaucuuuguagcucc

SEQ ID NO: 58 - RNA, 31 nt, Arabidopsis thaliana
uuggccuaauucuucuucugaugaucgauuc

SEQ ID NO: 59 - RNA, 31 nt, Arabidopsis thaliana
uccaaauaauuuaugcagcuucaacaucucc

SEQ ID NO: 60 - RNA, 31 nt, Arabidopsis thaliana
ucgguacaauccaaauaauuuaugcagcuuc

SEQ ID NO: 61 - RNA, 31 nt, Arabidopsis thaliana
uuggauuucuuauugcuuuugccgucaaauc

SEQ ID NO: 62 - RNA, 31 nt, Arabidopsis thaliana
uguuagcaauguacagcggucaaauaggauc

SEQ ID NO: 63 - RNA, 31 nt, Arabidopsis thaliana
cuuuggaccugguguaucuugucuuuaccac

SEQ ID NO: 64 - RNA, 31 nt, Arabidopsis thaliana
acuuuaucgauccacuuacuucuauuauguc

SEQ ID NO: 65 - RNA, 31 nt, Arabidopsis thaliana
uacaugauuuucuuuuaguuuuucugggauc

SEQ ID NO: 66 - RNA, 31 nt, Arabidopsis thaliana
aaaaacauauuuuauugagucccuucaugcc

SEQ ID NO: 67 - RNA, 31 nt, Arabidopsis thaliana
ggcauuccauuaauaacaggccguuuugauc

SEQ ID NO: 68 - RNA, 31 nt, Arabidopsis thaliana
cuguucauggacuagcuguaccuaccguuuc

SEQ ID NO: 69 - RNA, 31 nt, Arabidopsis thaliana
uggcaguuuuugcauuaauuauuacuucauc

SEQ ID NO: 70 - RNA, 31 nt, Arabidopsis thaliana
aucaauauacuuuuaaugucgaaucaggauc

SEQ ID NO: 71 - RNA, 31 nt, Arabidopsis thaliana
uagaaggaacauguauuacacgugcaaaauc

SEQ ID NO: 72 - RNA, 31 nt, Arabidopsis thaliana
auaacccagaaauaauucguguauauauuuc

SEQ ID NO: 73 - RNA, 31 nt, Arabidopsis thaliana
ggaaacaaaaaauaucuauucuaguucuauc

SEQ ID NO: 74 - RNA, 31 nt, Arabidopsis thaliana
acauuccuuuaaugaauucccuuggaacuuc

SEQ ID NO: 75 - RNA, 31 nt, Arabidopsis thaliana
aaaaaccuacuuucuuacgauuacgagguuc

SEQ ID NO: 76 - RNA, 31 nt, Arabidopsis thaliana
gacauaaaaaggaaauucuuuuugaaauauc

SEQ ID NO: 77 - RNA, 31 nt, Arabidopsis thaliana
aauggaaaauucauggaaaauuacaaucccc

SEQ ID NO: 78 - RNA, 31 nt, Arabidopsis thaliana
aaaaaaaauaucauuugauucgucgauccuc

SEQ ID NO: 79 - RNA, 31 nt, Arabidopsis thaliana
uuaucgcggaauuagaccugcuauuaacguc

SEQ ID NO: 80 - RNA, 31 nt, Arabidopsis thaliana
ugaaagcuaugaaacaaguaugcgguaguuc

SEQ ID NO: 81 - RNA, 31 nt, Arabidopsis thaliana
ucaauagaggugcaaggcugacagaaguacc

SEQ ID NO: 82 - RNA, 31 nt, Arabidopsis thaliana
acagaaucucucaauaugagaaagccauucc

SEQ ID NO: 83 - RNA, 31 nt, Arabidopsis thaliana
guggauuaacuaacgaaagaaaaauggaacc

SEQ ID NO: 84 - RNA, 31 nt, Arabidopsis thaliana
aucggaaacuucuauuucucauucacaaauc

SEQ ID NO: 85 - RNA, 31 nt, Arabidopsis thaliana
uggcgcgaaauccaucauuggcuaaacaauc

SEQ ID NO: 86 - RNA, 31 nt, Arabidopsis thaliana
cucuaaccgaagcuauugcauuguuugcccc

SEQ ID NO: 87 - RNA, 31 nt, Arabidopsis thaliana
cucaacccgagauguuagaaggugcaaaauc

SEQ ID NO: 88 - RNA, 31 nt, Arabidopsis thaliana
caauaggugccggagcugcuacaauugcuuc

SEQ ID NO: 89 - RNA, 31 nt, Arabidopsis thaliana
ccuuaaugcuagguuuugaaaaagacuuuuc

SEQ ID NO: 90 - RNA, 31 nt, Arabidopsis thaliana
uagguuuugaaaaagacuuuucaugucauuc

SEQ ID NO: 91 - RNA, 31 nt, Arabidopsis thaliana
aaagacuuuucaugucauucccauuuagguc

SEQ ID NO: 92 - RNA, 31 nt, Arabidopsis thaliana
aagacuuuucaugucauucccauuuaggucc

SEQ ID NO: 93 - RNA, 31 nt, Arabidopsis thaliana
uuuucaugucauucccauuuagguccgauuc

SEQ ID NO: 94 - RNA, 31 nt, Arabidopsis thaliana
augucauucccauuuagguccgauucggauc

SEQ ID NO: 95 - RNA, 31 nt, Arabidopsis thaliana
agaagaaguaaggaaaugagacgacuuuuuc

SEQ ID NO: 96 - RNA, 31 nt, Arabidopsis thaliana
ugucauucccauuuagguccgauucggaucc

SEQ ID NO: 97 - RNA, 31 nt, Arabidopsis thaliana
auucccauuuagguccgauucggaucccucc

SEQ ID NO: 98 - RNA, 31 nt, Arabidopsis thaliana
uuagguccgauucggaucccuccguuguuuc

SEQ ID NO: 99 - RNA, 31 nt, Arabidopsis thaliana
cgauucggaucccuccguuguuuccuuuucc

SEQ ID NO: 100 - RNA, 31 nt, Arabidopsis thaliana
auucggaucccuccguuguuuccuuuuccuc

SEQ ID NO: 101 - RNA, 31 nt, Arabidopsis thaliana
ucccuccguuguuuccuuuuccuccugcacc

SEQ ID NO: 102 - RNA, 31 nt, Arabidopsis thaliana
ccguuguuuccuuuuccuccugcaccuuuuc

SEQ ID NO: 103 - RNA, 31 nt, Arabidopsis thaliana
cguuguuuccuuuuccuccugcaccuuuucc

SEQ ID NO: 104 - RNA, 31 nt, Arabidopsis thaliana
gaaaugagacgacuuuuucuugaacuauauc

SEQ ID NO: 105 - RNA, 31 nt, Arabidopsis thaliana
aagauccuacuucuacaauuggugggucacc

SEQ ID NO: 106 - RNA, 31 nt, Arabidopsis thaliana
uuggugggucaccggguuauucaaauaaguc

SEQ ID NO: 107 - RNA, 31 nt, Arabidopsis thaliana
uuuucugugguuuucccauguuacaacuuuc

SEQ ID NO: 108 - RNA, 31 nt, Arabidopsis thaliana
ucguaccaauucggucgauccggaauggauc

SEQ ID NO: 109 - RNA, 31 nt, Arabidopsis thaliana
ggucgauccggaauggaucgguuaaacauuc

SEQ ID NO: 110 - RNA, 31 nt, Arabidopsis thaliana
gucgauccggaauggaucgguuaaacauucc

SEQ ID NO: 111 - RNA, 31 nt, Arabidopsis thaliana
auuccauuagggagccuggucuugacucuuc

SEQ ID NO: 112 - RNA, 31 nt, Arabidopsis thaliana
gucuugacucuucugugugguauucauucuc

SEQ ID NO: 113 - RNA, 31 nt, Arabidopsis thaliana
ugacucuucugugugguauucauucucguuc

SEQ ID NO: 114 - RNA, 31 nt, Arabidopsis thaliana
gaaucacauccagcagugguuggaacagcuc

SEQ ID NO: 115 - RNA, 31 nt, Arabidopsis thaliana
uccagcagugguuggaacagcucgcaaaauc

SEQ ID NO: 116 - RNA, 31 nt, Arabidopsis thaliana
ccagcagugguuggaacagcucgcaaaaucc

SEQ ID NO: 117 - RNA, 31 nt, Arabidopsis thaliana
guuggaacagcucgcaaaauccaaccacuuc

SEQ ID NO: 118 - RNA, 31 nt, Arabidopsis thaliana
cuucaccuacuuuauugccccuaaccguuuc

SEQ ID NO: 119 - RNA, 31 nt, Arabidopsis thaliana
ucaccuacuuuauugccccuaaccguuucuc

SEQ ID NO: 120 - RNA, 31 nt, Arabidopsis thaliana
cuauugaaacagaaugguuucauguucuuuc

SEQ ID NO: 121 - RNA, 31 nt, Arabidopsis thaliana
uugaaacagaaugguuucauguucuuucauc

SEQ ID NO: 122 - RNA, 31 nt, Arabidopsis thaliana
gguuucauguucuuucaucgauugguuauuc

SEQ ID NO: 123 - RNA, 31 nt, Arabidopsis thaliana
uucauguucuuucaucgauugguuauuccuc

SEQ ID NO: 124 - RNA, 31 nt, Arabidopsis thaliana
ucuccuccacaccaaucacgaguuuuucuuc

SEQ ID NO: 125 - RNA, 31 nt, Arabidopsis thaliana
cuccacaccaaucacgaguuuuucuucauuc

SEQ ID NO: 126 - RNA, 31 nt, Arabidopsis thaliana
cacaccaaucacgaguuuuucuucauuccuc

SEQ ID NO: 127 - RNA, 31 nt, Arabidopsis thaliana
caccaaucacgaguuuuucuucauuccucuc

SEQ ID NO: 128 - RNA, 31 nt, Arabidopsis thaliana
ucuugguuguucuuaacagcgauggcuauuc

SEQ ID NO: 129 - RNA, 31 nt, Arabidopsis thaliana
cauuuaagucuugggguagcaccacuagauc

SEQ ID NO: 130 - RNA, 31 nt, Arabidopsis thaliana
auucucguauucucuauguacauguuccugc

SEQ ID NO: 131 - RNA, 31 nt, Arabidopsis thaliana
cguauucucuauguacauguuccugcggcuc

SEQ ID NO: 132 - RNA, 31 nt, Arabidopsis thaliana
uuccuauuaacaaaacauccccuuuaucuuc

SEQ ID NO: 133 - RNA, 31 nt, Arabidopsis thaliana
acguuguuuaccuuaguuacugggggguuuc

SEQ ID NO: 134 - RNA, 31 nt, Arabidopsis thaliana
gggaugcucguuugaccucuguauucaucuc

SEQ ID NO: 135 - RNA, 31 nt, Arabidopsis thaliana
gcucguuugaccucuguauucaucucguuuc

SEQ ID NO: 136 - RNA, 31 nt, Arabidopsis thaliana
aucucguuucuuauuuaccugggugcacugc

SEQ ID NO: 137 - RNA, 31 nt, Arabidopsis thaliana
cacugcguuuucaaaagcuuccugucgaacc

SEQ ID NO: 138 - RNA, 31 nt, Arabidopsis thaliana
aaaagcuuccugucgaaccggcuucuauuuc

SEQ ID NO: 139 - RNA, 31 nt, Arabidopsis thaliana
cuuccugucgaaccggcuucuauuucaauuc

SEQ ID NO: 140 - RNA, 31 nt, Arabidopsis thaliana
cugucgaaccggcuucuauuucaauucgugc

SEQ ID NO: 141 - RNA, 31 nt, Arabidopsis thaliana
aaccggcuucuauuucaauucgugcuggacc

SEQ ID NO: 142 - RNA, 31 nt, Arabidopsis thaliana
ggcuucuauuucaauucgugcuggaccgauc

SEQ ID NO: 143 - RNA, 31 nt, Arabidopsis thaliana
cuggaccgaucgauauaccaauaauaaaguc

SEQ ID NO: 144 - RNA, 31 nt, Arabidopsis thaliana
uaaagucuucagucaacugguggaauacauc

SEQ ID NO: 145 - RNA, 31 nt, Arabidopsis thaliana
caucgcaucaaccugggagcauuagccgauc

SEQ ID NO: 146 - RNA, 31 nt, Arabidopsis thaliana
auuagccgaucugguacaucaauacauguuc

SEQ ID NO: 147 - RNA, 31 nt, Arabidopsis thaliana
gaucugguacaucaauacauguuccuaugcc

SEQ ID NO: 148 - RNA, 31 nt, Arabidopsis thaliana
uuccaaucuugucuaacuuugcuaacuuccc

SEQ ID NO: 149 - RNA, 31 nt, Arabidopsis thaliana
ucuugucuaacuuugcuaacuuccccuucuc

SEQ ID NO: 150 - RNA, 31 nt, Arabidopsis thaliana
gucuaacuuugcuaacuuccccuucucaacc

SEQ ID NO: 151 - RNA, 31 nt, Arabidopsis thaliana
ucuaacuuugcuaacuuccccuucucaaccc

SEQ ID NO: 152 - RNA, 31 nt, Arabidopsis thaliana
cuuugcuaacuuccccuucucaacccguauc

SEQ ID NO: 153 - RNA, 31 nt, Arabidopsis thaliana
guaucuuguuuguucuggaaacacgucuucc

SEQ ID NO: 154 - RNA, 31 nt, Arabidopsis thaliana
uguuuguucuggaaacacgucuuccuauucc

SEQ ID NO: 155 - RNA, 31 nt, Arabidopsis thaliana
cgucuuccuauuccaucuuuucucgaaucuc

SEQ ID NO: 156 - RNA, 31 nt, Arabidopsis thaliana
cuauugaaaugguucgucaguagagauguuc

SEQ ID NO: 157 - RNA, 31 nt, Arabidopsis thaliana
agcacggcugaaguggcuauacauacaaauc

SEQ ID NO: 158 - RNA, 31 nt, Arabidopsis thaliana
auacaaaucuauuuacggaucuauaugcuuc

SEQ ID NO: 159 - RNA, 31 nt, Arabidopsis thaliana
aaguuccagaacaggagguugguauaccacc

SEQ ID NO: 160 - RNA, 31 nt, Arabidopsis thaliana
guagagauguucccacgggugccccuuuuuc

SEQ ID NO: 161 - RNA, 31 nt, Arabidopsis thaliana
uagagauguucccacgggugccccuuuuucc

SEQ ID NO: 162 - RNA, 31 nt, Arabidopsis thaliana
auaaugaaacugccuuuuauuuuuuuuauuc

SEQ ID NO: 163 - RNA, 31 nt, Arabidopsis thaliana
uaggauuuauguuggcuucguugggaggcuc

SEQ ID NO: 164 - RNA, 31 nt, Arabidopsis thaliana
cagcuccaaaaggauaaguugcguuggaauc

SEQ ID NO: 165 - RNA, 31 nt, Arabidopsis thaliana
cuuuuuccaaugguacuauaauuccuauucc

SEQ ID NO: 166 - RNA, 31 nt, Arabidopsis thaliana
augguacuauaauuccuauuccuaucucuuc

SEQ ID NO: 167 - RNA, 31 nt, Arabidopsis thaliana
acuauaauuccuauuccuaucucuucauucc

SEQ ID NO: 168 - RNA, 31 nt, Arabidopsis thaliana
ccuaucucuucauucccucuuuuggucuauc

SEQ ID NO: 169 - RNA, 31 nt, Arabidopsis thaliana
cuuauuuuuuuucguucccguucuucauuuc

SEQ ID NO: 170 - RNA, 31 nt, Arabidopsis thaliana
uuauuuuuuuucguucccguucuucauuucc

SEQ ID NO: 171 - RNA, 31 nt, Arabidopsis thaliana
caagggggacuucucauauuuagaaucuuuc

SEQ ID NO: 172 - RNA, 31 nt, Arabidopsis thaliana
uucugcggugugcucuguuuacuauucuuuc

SEQ ID NO: 173 - RNA, 31 nt, Arabidopsis thaliana
gugcucuguuuacuauucuuucguacuuucc

SEQ ID NO: 174 - RNA, 31 nt, Arabidopsis thaliana
uuuucuuuuuuauuauuuuuauggucgugcc

SEQ ID NO: 175 - RNA, 31 nt, Arabidopsis thaliana
gcacccccauuuagauuuagaaagaaggguc

SEQ ID NO: 176 - RNA, 31 nt, Arabidopsis thaliana
uccauuugugggaauuugaugaucuauaaac

SEQ ID NO: 177 - RNA, 31 nt, Arabidopsis thaliana
agaaacaaccaccagcguuuggugcagcacc

SEQ ID NO: 178 - RNA, 31 nt, Arabidopsis thaliana
ggugcauucuucuuucuuuccuuggucuuuc

SEQ ID NO: 179 - RNA, 31 nt, Arabidopsis thaliana
ucuuuccuuggucuuucguucugucauauuc

SEQ ID NO: 180 - RNA, 31 nt, Arabidopsis thaliana
ccaauuacaacguauuaaccgcuaaugcacc

SEQ ID NO: 181 - RNA, 31 nt, Arabidopsis thaliana
aaucaugaggguaguauuuuauuaugguguc

SEQ ID NO: 182 - RNA, 31 nt, Arabidopsis thaliana
aggguaguauuuuauuauggugucggauccc

SEQ ID NO: 183 - RNA, 31 nt, Arabidopsis thaliana
ugucggaucccaaauuuuuauggauuuuuuc

SEQ ID NO: 184 - RNA, 31 nt, Arabidopsis thaliana
cagagccauaaugucuuaaaacaaggaggcc

SEQ ID NO: 185 - RNA, 31 nt, Arabidopsis thaliana
auagggaaagucuuuuuuuuuuuuuugucuc

SEQ ID NO: 186 - RNA, 31 nt, Arabidopsis thaliana
aagucuuuuuuuuuuuuuugucucgaacuuc

SEQ ID NO: 187 - RNA, 31 nt, Arabidopsis thaliana
acuucgugaagaacucaauuuuaucucuccc

SEQ ID NO: 188 - RNA, 31 nt, Arabidopsis thaliana
uauaugaauucuuucauuauucguuauuucc

SEQ ID NO: 189 - RNA, 31 nt, Arabidopsis thaliana
guucuacgaacccuuguugauucugaacuuc

SEQ ID NO: 190 - RNA, 31 nt, Arabidopsis thaliana
gaaaauuaaaaauccucuggacgcuuggcgc

SEQ ID NO: 191 - RNA, 31 nt, Arabidopsis thaliana
aaauuaaaaauccucuggacgcuuggcgcuc

SEQ ID NO: 192 - RNA, 31 nt, Arabidopsis thaliana
ggagcucuuggcauugcuuuguuuuucucuc

SEQ ID NO: 193 - RNA, 31 nt, Arabidopsis thaliana
gagcucuuggcauugcuuuguuuuucucucc

SEQ ID NO: 194 - RNA, 31 nt, Arabidopsis thaliana
gcauugcuuuguuuuucucuccuuuccuauc

SEQ ID NO: 195 - RNA, 31 nt, Arabidopsis thaliana
ucuuuguuuguaccgaaccgcuugcagaauc

SEQ ID NO: 196 - RNA, 31 nt, Arabidopsis thaliana
ccgaaccgcuugcagaaucaaauccuguucc

SEQ ID NO: 197 - RNA, 31 nt, Arabidopsis thaliana
aaucaaauccuguuccacaagauccuauauc

SEQ ID NO: 198 - RNA, 31 nt, Arabidopsis thaliana
gaugccgccgaaaagaauggaacgcugcuuc

SEQ ID NO: 199 - RNA, 31 nt, Arabidopsis thaliana
guuggugguuuuuaaccguaggcaucuugcc

SEQ ID NO: 200 - RNA, 31 nt, Arabidopsis thaliana
ggaaguuggugggcuuaucaugaauuagguc

SEQ ID NO: 201 - RNA, 31 nt, Arabidopsis thaliana
caugaauuaggucgggguggcuggugguuuc

SEQ ID NO: 202 - RNA, 31 nt, Arabidopsis thaliana
gaucccguagaaaaugcuucuuuuaugccuc

SEQ ID NO: 203 - RNA, 31 nt, Arabidopsis thaliana
ucuuuuaugccucggguauuagccacagcuc

SEQ ID NO: 204 - RNA, 31 nt, Arabidopsis thaliana
acagcucguauucauucuguaauuuuacccc

SEQ ID NO: 205 - RNA, 31 nt, Arabidopsis thaliana
uaauuuuaccccuucuucauucuuggaccuc

SEQ ID NO: 206 - RNA, 31 nt, Arabidopsis thaliana
ggaccucguuucuuaauauugugacuuuucc

SEQ ID NO: 207 - RNA, 31 nt, Arabidopsis thaliana
uuaauauugugacuuuuccaugcugugucuc

SEQ ID NO: 208 - RNA, 31 nt, Arabidopsis thaliana
accuuuucaauacgguccggauugcuagcuc

SEQ ID NO: 209 - RNA, 31 nt, Arabidopsis thaliana
ggugguucuuccuucuaaugaccggcauauc

SEQ ID NO: 210 - RNA, 31 nt, Arabidopsis thaliana
uucguaauggaaagaaagagaccacuacuuc

SEQ ID NO: 211 - RNA, 31 nt, Arabidopsis thaliana
agacuuacaucacgauaucuuuuucuuccuc

SEQ ID NO: 212 - RNA, 31 nt, Arabidopsis thaliana
uuugaaaaugauuguucuaaaaugguuauuc

SEQ ID NO: 213 - RNA, 31 nt, Arabidopsis thaliana
uugaaaaugauuguucuaaaaugguuauucc

SEQ ID NO: 214 - RNA, 31 nt, Arabidopsis thaliana
auuguucauggaacuacuaucgagauucuuc

SEQ ID NO: 215 - RNA, 31 nt, Arabidopsis thaliana
uggaacuacuaucgagauucuucggaccauc

SEQ ID NO: 216 - RNA, 31 nt, Arabidopsis thaliana
gaaaaugauuguucuaaaaugguuauuccuc

SEQ ID NO: 217 - RNA, 31 nt, Arabidopsis thaliana
uucuucggaccaucuuuccuaguaucaucuc

SEQ ID NO: 218 - RNA, 31 nt, Arabidopsis thaliana
acuaucaaagcuauuggacaucaaugguauc

SEQ ID NO: 219 - RNA, 31 nt, Arabidopsis thaliana
uuccagaagaagaucuagaauugggucaauc

SEQ ID NO: 220 - RNA, 31 nt, Arabidopsis thaliana
uacguauuauuguaacaucugcugauguacc

SEQ ID NO: 221 - RNA, 31 nt, Arabidopsis thaliana
auguaccucauaguugggcuguaccuuccuc

SEQ ID NO: 222 - RNA, 31 nt, Arabidopsis thaliana
gugagauuuguggaacuaaucaugccuuuac

SEQ ID NO: 223 - RNA, 31 nt, Arabidopsis thaliana
gugaugcagcggaaccauggcaauuaggauc

SEQ ID NO: 224 - RNA, 31 nt, Arabidopsis thaliana
gccuuuacgucuaucgucguagaagcuguuc

SEQ ID NO: 225 - RNA, 31 nt, Arabidopsis thaliana
gaagcuguuccuaggaaagauuaugguucuc

SEQ ID NO: 226 - RNA, 31 nt, Arabidopsis thaliana
accaccguaggaggugugauguacaugcacc

SEQ ID NO: 227 - RNA, 31 nt, Arabidopsis thaliana
gacaucauaccaaagucguacaauuaggacc

SEQ ID NO: 228 - RNA, 31 nt, Arabidopsis thaliana
aagucguacaauuaggaccucgauaugguuc

SEQ ID NO: 229 - RNA, 31 nt, Arabidopsis thaliana
uuauguucuuuuuugcuuuuuuuugggcuuc

SEQ ID NO: 230 - RNA, 31 nt, Arabidopsis thaliana
uguucuuuuuugcuuuuuuuugggcuucuuc

SEQ ID NO: 231 - RNA, 31 nt, Arabidopsis thaliana
auccuugggaaaucccuuuucuuaauacccc

SEQ ID NO: 232 - RNA, 31 nt, Arabidopsis thaliana
aaaucccuuuucuuaauaccccuauucuccc

SEQ ID NO: 233 - RNA, 31 nt, Arabidopsis thaliana
uucggauaguauuuaugguucuaccuuuuuc

SEQ ID NO: 234 - RNA, 31 nt, Arabidopsis thaliana
gcuccauuuguuacuauuggacaaauuucuc

SEQ ID NO: 235 - RNA, 31 nt, Arabidopsis thaliana
agcaaucuuaguuauugguggggguucgguc

SEQ ID NO: 236 - RNA, 31 nt, Arabidopsis thaliana
uauaugcaugcuaauggggcaaguauguuuc

SEQ ID NO: 237 - RNA, 31 nt, Arabidopsis thaliana
guuuaccuucauauuuuucguggucuauauc

SEQ ID NO: 238 - RNA, 31 nt, Arabidopsis thaliana
gccaccuuaaaucguuuuuuuagucuucauc

SEQ ID NO: 239 - RNA, 31 nt, Arabidopsis thaliana
uuuauuuuaguaggcgccagucuucuucauc

SEQ ID NO: 240 - RNA, 31 nt, Arabidopsis thaliana
auugugccggaaugguauuuccuaccgaucc

SEQ ID NO: 241 - RNA, 31 nt, Arabidopsis thaliana
acaaagcgggagguguagccgcaauagcacc

SEQ ID NO: 242 - RNA, 31 nt, Arabidopsis thaliana
agccgcaauagcaccaguuuuuauaugucuc

SEQ ID NO: 243 - RNA, 31 nt, Arabidopsis thaliana
uaugugcguaguucaaguuuucgaccgauuc

SEQ ID NO: 244 - RNA, 31 nt, Arabidopsis thaliana
acacugggcgggaucuaucagcagcgaauuc

SEQ ID NO: 245 - RNA, 31 nt, Arabidopsis thaliana
cugggcgggaucuaucagcagcgaauucccc

SEQ ID NO: 246 - RNA, 31 nt, Arabidopsis thaliana
gagguaucauuagccgaagaagacccuggcc

SEQ ID NO: 247 - RNA, 31 nt, Arabidopsis thaliana
acgucagcgacgaagacaucguaaauugguc

SEQ ID NO: 248 - RNA, 31 nt, Arabidopsis thaliana
cgucagcgacgaagacaucguaaauuggucc

SEQ ID NO: 249 - RNA, 31 nt, Arabidopsis thaliana
uaaauugguccgcgggcaucgcgauaagucc

SEQ ID NO: 250 - RNA, 31 nt, Arabidopsis thaliana
gcgauaaguccucuguccuacuacaggugcc

SEQ ID NO: 251 - RNA, 31 nt, Arabidopsis thaliana
aaccuuuaucaaguccgaacgauugucgacc

SEQ ID NO: 252 - RNA, 31 nt, Arabidopsis thaliana
cgaauauaauccucaaguacuccaaagacuc

SEQ ID NO: 253 - RNA, 31 nt, Arabidopsis thaliana
uuucacaccaucgaccgacaucgacucaucc

SEQ ID NO: 254 - RNA, 31 nt, Arabidopsis thaliana
aagagaucgacgaucccaaguucuuuuacuc

SEQ ID NO: 255 - RNA, 31 nt, Arabidopsis thaliana
ucccacacaguguacuacuaucggcccuacc

SEQ ID NO: 256 - RNA, 31 nt, Arabidopsis thaliana
acgaaauuccgauuguucagagagucagauc

SEQ ID NO: 257 - RNA, 31 nt, Arabidopsis thaliana
ugaaagaggcgaucagaaugguacucgaauc

SEQ ID NO: 258 - RNA, 31 nt, Arabidopsis thaliana
ucggauuguuacaaccucuagcagaugguuc

SEQ ID NO: 259 - RNA, 31 nt, Arabidopsis thaliana
ccagaucaugaguaaauaaaaaaucgaaaac

SEQ ID NO: 260 - RNA, 31 nt, Arabidopsis thaliana
guggcuacauuuauguuaagucuggucgcuc

SEQ ID NO: 261 - RNA, 31 nt, Arabidopsis thaliana
ccuuuugauuaugguaugguauugucagauc

SEQ ID NO: 262 - RNA, 31 nt, Arabidopsis thaliana
cuuuugauuaugguaugguauugucagaucc

SEQ ID NO: 263 - RNA, 31 nt, Arabidopsis thaliana
cuagguguuuauggaauuauuauagcggguc

SEQ ID NO: 264 - RNA, 31 nt, Arabidopsis thaliana
auucuuauuacuguacuaauauguguagguc

SEQ ID NO: 265 - RNA, 31 nt, Arabidopsis thaliana
ucuuauuacuguacuaauauguguagguccc

SEQ ID NO: 266 - RNA, 31 nt, Arabidopsis thaliana
cuuauuacuguacuaauauguguaggucccc

SEQ ID NO: 267 - RNA, 31 nt, Arabidopsis thaliana
cuguacuaauauguguagguccccguaauuc

SEQ ID NO: 268 - RNA, 31 nt, Arabidopsis thaliana
agauugucauggcgcaaaagcagauaugguc

SEQ ID NO: 269 - RNA, 31 nt, Arabidopsis thaliana
ggcgcaaaagcagauauggucugguauuccc

SEQ ID NO: 270 - RNA, 31 nt, Arabidopsis thaliana
auuccccuguucccuguauugguuauguucc

SEQ ID NO: 271 - RNA, 31 nt, Arabidopsis thaliana
uucccuguauugguuauguuccuuauuucuc

SEQ ID NO: 272 - RNA, 31 nt, Arabidopsis thaliana
cguuugaucucccagaagcggaagcugaauc

SEQ ID NO: 273 - RNA, 31 nt, Arabidopsis thaliana
gcuauaauguagaauauucuucaaugggguc

SEQ ID NO: 274 - RNA, 31 nt, Arabidopsis thaliana
aguaugccaauaugaucuuaaugaguggucc

SEQ ID NO: 275 - RNA, 31 nt, Arabidopsis thaliana
uaaugagugguccaugcacauuguucuuucc

SEQ ID NO: 276 - RNA, 31 nt, Arabidopsis thaliana
caugcacauuguucuuuccaggagguuggcc

SEQ ID NO: 277 - RNA, 31 nt, Arabidopsis thaliana
uuguucuuuccaggagguuggccgccuaucc

SEQ ID NO: 278 - RNA, 31 nt, Arabidopsis thaliana
aucuucccauuuucaagaagaucccgggcuc

SEQ ID NO: 279 - RNA, 31 nt, Arabidopsis thaliana
ggcucgaucugguuuaguaucaagguucuuc

SEQ ID NO: 280 - RNA, 31 nt, Arabidopsis thaliana
uaucguuaugaucaauuaaugggacuuggcc

SEQ ID NO: 281 - RNA, 31 nt, Arabidopsis thaliana
cggaaaguguucuugccucuaucauuagcuc

SEQ ID NO: 282 - RNA, 31 nt, Arabidopsis thaliana
uucuugccucuaucauuagcucggguagucc

SEQ ID NO: 283 - RNA, 31 nt, Arabidopsis thaliana
uaaugacgauggaugcauucgccauaguuuc

SEQ ID NO: 284 - RNA, 31 nt, Arabidopsis thaliana
ugggcgcucuagccaaaacgaauccuauuuc

SEQ ID NO: 285 - RNA, 31 nt, Arabidopsis thaliana
acccccguuagccggcuuuuguagcaaauuc

SEQ ID NO: 286 - RNA, 31 nt, Arabidopsis thaliana
gcuuuggguuguggggcuuacuuucuagccc

SEQ ID NO: 287 - RNA, 31 nt, Arabidopsis thaliana
cuuuggguuguggggcuuacuuucuagcccc

SEQ ID NO: 288 - RNA, 31 nt, Arabidopsis thaliana
ccagugggaguagugacuagcguuauagguc

SEQ ID NO: 289 - RNA, 31 nt, Arabidopsis thaliana
uacuagcaaugacuuccuuuuucauuacuuc

SEQ ID NO: 290 - RNA, 31 nt, Arabidopsis thaliana
uagcaaugacuuccuuuuucauuacuucauc

SEQ ID NO: 291 - RNA, 31 nt, Arabidopsis thaliana
ucucaguuacucaucaaauggcacucaguuc

SEQ ID NO: 292 - RNA, 31 nt, Arabidopsis thaliana
ucuuuuuaggagggacaauuuuacauauuuc

SEQ ID NO: 293 - RNA, 31 nt, Arabidopsis thaliana
cggcugguaccauuucgauguguuucgauuc

SEQ ID NO: 294 - RNA, 31 nt, Arabidopsis thaliana
cugguaccauuucgauguguuucgauucuuc

SEQ ID NO: 295 - RNA, 31 nt, Arabidopsis thaliana
uugaugcuuuugaauucauuguauuaauucc

SEQ ID NO: 296 - RNA, 31 nt, Arabidopsis thaliana
gcuuuugaauucauuguauuaauuccacuuc

SEQ ID NO: 297 - RNA, 31 nt, Arabidopsis thaliana
gaauucauuguauuaauuccacuuccuacuc

SEQ ID NO: 298 - RNA, 31 nt, Arabidopsis thaliana
acucgcgguaugcucuuuaugaucucggcuc

SEQ ID NO: 299 - RNA, 31 nt, Arabidopsis thaliana
cuuuaugaucucggcucaugauuuaauugcc

SEQ ID NO: 300 - RNA, 31 nt, Arabidopsis thaliana
auuuaauugccauguauuuagcuauugagcc

SEQ ID NO: 301 - RNA, 31 nt, Arabidopsis thaliana
aagaaagucugaauuuuccacggaagccggc

SEQ ID NO: 302 - RNA, 31 nt, Arabidopsis thaliana
gaaagucugaauuuuccacggaagccggcuc

SEQ ID NO: 303 - RNA, 31 nt, Arabidopsis thaliana
cucgaaauauuugaucuuaggugcauuuucc

SEQ ID NO: 304 - RNA, 31 nt, Arabidopsis thaliana
uuccucuggaauauuauuguuugguuguucc

SEQ ID NO: 305 - RNA, 31 nt, Arabidopsis thaliana
cacacauguucaaucuuuuuuuagcgguuuc

SEQ ID NO: 306 - RNA, 31 nt, Arabidopsis thaliana
ccacuucgaucaauuagccaagauuuugacc

SEQ ID NO: 307 - RNA, 31 nt, Arabidopsis thaliana
gaucuagugguauuuuuauggggauucuguc

SEQ ID NO: 308 - RNA, 31 nt, Arabidopsis thaliana
uccuuucuauugcgccuaaaaucucuauuuc

SEQ ID NO: 309 - RNA, 31 nt, Arabidopsis thaliana
ucucuauuucugcuaauauuuuacguguuuc

SEQ ID NO: 310 - RNA, 31 nt, Arabidopsis thaliana
ccccagagaucuuuaucauuaaugcaaccuc

SEQ ID NO: 311 - RNA, 31 nt, Arabidopsis thaliana
cccagagaucuuuaucauuaaugcaaccucc

SEQ ID NO: 312 - RNA, 31 nt, Arabidopsis thaliana
ccgccauggcccaaacgaaagucaaaagacc

SEQ ID NO: 313 - RNA, 31 nt, Arabidopsis thaliana
gcccaaacgaaagucaaaagaccucuagcuc

SEQ ID NO: 314 - RNA, 31 nt, Arabidopsis thaliana
cauaguucaauuggacauguagguuauauuc

SEQ ID NO: 315 - RNA, 31 nt, Arabidopsis thaliana
guucaauuggacauguagguuauauucguac

SEQ ID NO: 316 - RNA, 31 nt, Arabidopsis thaliana
ugucggccuacgaaugugguuucgauccuuc

SEQ ID NO: 317 - RNA, 31 nt, Arabidopsis thaliana
uuuuaucuuguuucaauuuuauuuuuaaucc

SEQ ID NO: 318 - RNA, 31 nt, Arabidopsis thaliana
uuuaucuuguuucaauuuuauuuuuaauccc

SEQ ID NO: 319 - RNA, 31 nt, Arabidopsis thaliana
gaaguaaccuuuuucuuuccuugggcaguac

SEQ ID NO: 320 - RNA, 31 nt, Arabidopsis thaliana
uaaccuuuuucuuuccuugggcaguaccucc

SEQ ID NO: 321 - RNA, 31 nt, Arabidopsis thaliana
cuguaaugaugucagaauuugcaccaauuuc

SEQ ID NO: 322 - RNA, 31 nt, Arabidopsis thaliana
gauuucuauaugaauggaaaaggggugcuuc

SEQ ID NO: 323 - RNA, 31 nt, Arabidopsis thaliana
cuauaugaauggaaaaggggugcuucggauc

SEQ ID NO: 324 - RNA, 31 nt, Arabidopsis thaliana
uuagugauuagucugcuaguuucuuugaucc

SEQ ID NO: 325 - RNA, 31 nt, Arabidopsis thaliana
gauuagucugcuaguuucuuugauccuacuc

SEQ ID NO: 326 - RNA, 31 nt, Arabidopsis thaliana
gcgagaaaacaaagugggcuguaaugauguc

SEQ ID NO: 327 - RNA, 31 nt, Arabidopsis thaliana
uuucuuugauccuacucgguguuccuuuucc

SEQ ID NO: 328 - RNA, 31 nt, Arabidopsis thaliana
acauacagggaauuggagguagcauucuacc

SEQ ID NO: 329 - RNA, 31 nt, Arabidopsis thaliana
auucuaccgauguuaagucauggacugguuc

SEQ ID NO: 330 - RNA, 31 nt, Arabidopsis thaliana
uucuuuucauuccaaauucaagaauacgacc

SEQ ID NO: 331 - RNA, 31 nt, Arabidopsis thaliana
ccgacauaagacucgacuuguuagauauuac

SEQ ID NO: 332 - RNA, 31 nt, Arabidopsis thaliana
uacggagguuuagugagcaccaugccgaauc

SEQ ID NO: 333 - RNA, 31 nt, Arabidopsis thaliana
cggagguuuagugagcaccaugccgaaucuc

SEQ ID NO: 334 - RNA, 31 nt, Arabidopsis thaliana
gagguuuagugagcaccaugccgaaucucuc

SEQ ID NO: 335 - RNA, 31 nt, Arabidopsis thaliana
ccaugccgaaucucucuaccauuuucuuuuc

SEQ ID NO: 336 - RNA, 31 nt, Arabidopsis thaliana
ucuuuucuuuuacuuuggccaauaugaguuc

SEQ ID NO: 337 - RNA, 31 nt, Arabidopsis thaliana
ugguacuagcagcuuuaucggggaauuucuc

SEQ ID NO: 338 - RNA, 31 nt, Arabidopsis thaliana
ucaagaauacgaccgauacgauuaauugguc

SEQ ID NO: 339 - RNA, 31 nt, Arabidopsis thaliana
aaccugauuuccuccauaaauucuccgauuc

SEQ ID NO: 340 - RNA, 31 nt, Arabidopsis thaliana
aauucuccgauucaaauggcagagaaguuuc

SEQ ID NO: 341 - RNA, 31 nt, Arabidopsis thaliana
uuccauauuuauaccuuuucuuguuggacuc

SEQ ID NO: 342 - RNA, 31 nt, Arabidopsis thaliana
auauuuauaccuuuucuuguuggacucguuc

SEQ ID NO: 343 - RNA, 31 nt, Arabidopsis thaliana
uuucuuguuggacucguucggauggguguuc

SEQ ID NO: 344 - RNA, 31 nt, Arabidopsis thaliana
uucggauggguguucaccccaaaguguuccc

SEQ ID NO: 345 - RNA, 31 nt, Arabidopsis thaliana
gugccucucuuauuacuuuuuuguauucucc

SEQ ID NO: 346 - RNA, 31 nt, Arabidopsis thaliana
cucuuauuacuuuuuuguauucuccuguucc

SEQ ID NO: 347 - RNA, 31 nt, Arabidopsis thaliana
cuuauuacuuuuuuguauucuccuguuccuc

SEQ ID NO: 348 - RNA, 31 nt, Arabidopsis thaliana
ggauacaauucgacucuucuacggccaaauc

SEQ ID NO: 349 - RNA, 31 nt, Arabidopsis thaliana
cuauguuagaacauuucugugaaugcuauuc

SEQ ID NO: 350 - RNA, 31 nt, Arabidopsis thaliana
ugaccacauuucugaucccuauuugcauuuc

SEQ ID NO: 351 - RNA, 31 nt, Arabidopsis thaliana
guaugagaaguuaugggaaagaguauauuac

SEQ ID NO: 352 - RNA, 31 nt, Arabidopsis thaliana
gggaaagaguauauuacagcauuuuuaauuc

SEQ ID NO: 353 - RNA, 31 nt, Arabidopsis thaliana
aauucgugaauuucuaaugaucgccguguuc

SEQ ID NO: 354 - RNA, 31 nt, Arabidopsis thaliana
auucgugaauuucuaaugaucgccguguucc

SEQ ID NO: 355 - RNA, 31 nt, Arabidopsis thaliana
augaucgccguguuccgcaugcuagaucuuc

SEQ ID NO: 356 - RNA, 31 nt, Arabidopsis thaliana
augcuagaucuucuacuauucuauguuuuuc

SEQ ID NO: 357 - RNA, 31 nt, Arabidopsis thaliana
ugcuagaucuucuacuauucuauguuuuucc

SEQ ID NO: 358 - RNA, 31 nt, Arabidopsis thaliana
uacuauucuauguuuuucccgaaagcgugcc

SEQ ID NO: 359 - RNA, 31 nt, Arabidopsis thaliana
uccaaacaggaaccaccgauuuacaaauauc

SEQ ID NO: 360 - RNA, 31 nt, Arabidopsis thaliana
agcggcgccaaaucuuucuauggauugcuuc

SEQ ID NO: 361 - RNA, 31 nt, Arabidopsis thaliana
uuauucuguguccugugcuaggaagcauuac

SEQ ID NO: 362 - RNA, 31 nt, Arabidopsis thaliana
cggcaggauccgucaucuuggcaggaauucc

SEQ ID NO: 363 - RNA, 31 nt, Arabidopsis thaliana
uuggcaggaauuccuuuaaaauuuggaaccc

SEQ ID NO: 364 - RNA, 31 nt, Arabidopsis thaliana
uacccauguuucccgaagcgacacuuuguuc

SEQ ID NO: 365 - RNA, 31 nt, Arabidopsis thaliana
uccugugcuaggaagcauuacucuucuuuuc

SEQ ID NO: 366 - RNA, 31 nt, Arabidopsis thaliana
uugcuauaauauauacuuccuugaccacuuc

SEQ ID NO: 367 - RNA, 31 nt, Arabidopsis thaliana
ugaaucuggugacuauugguauguuuagucc

SEQ ID NO: 368 - RNA, 31 nt, Arabidopsis thaliana
aauagacgaaauauuccuauuaugucaaugc

SEQ ID NO: 369 - RNA, 31 nt, Arabidopsis thaliana
auauuccuauuaugucaaugccaauugaauc

SEQ ID NO: 370 - RNA, 31 nt, Arabidopsis thaliana
caauugaaucaauguuauuagcugugaauuc

SEQ ID NO: 371 - RNA, 31 nt, Arabidopsis thaliana
auucgaacuuuuugguauuuuccguuucuuc

SEQ ID NO: 372 - RNA, 31 nt, Arabidopsis thaliana
cggaugauaugaugggucaaguauuugcuuc

SEQ ID NO: 373 - RNA, 31 nt, Arabidopsis thaliana
ugaugggucaaguauuugcuucauugguucc

SEQ ID NO: 374 - RNA, 31 nt, Arabidopsis thaliana
ucaaauauuucacauuuucuaugauuauuuc

SEQ ID NO: 375 - RNA, 31 nt, Arabidopsis thaliana
uuuucuaugauuauuucuauuuuagguauuc

SEQ ID NO: 376 - RNA, 31 nt, Arabidopsis thaliana
ggggaauccuccuuaauagacgaaauauucc

SEQ ID NO: 377 - RNA, 31 nt, Arabidopsis thaliana
uccuuaauagacgaaauauuccuauuauguc

SEQ ID NO: 378 - RNA, 31 nt, Arabidopsis thaliana
ugggaacuuugcuuucugguugggaaguguc

SEQ ID NO: 379 - RNA, 31 nt, Arabidopsis thaliana
guuuagguaccaauuuuugggccaauucccc

SEQ ID NO: 380 - RNA, 31 nt, Arabidopsis thaliana
uaucuuugauugcuuuuuaugaagucgcacc

SEQ ID NO: 381 - RNA, 31 nt, Arabidopsis thaliana
ccgaauccgaguuugcugcuccaaccauuac

SEQ ID NO: 382 - RNA, 31 nt, Arabidopsis thaliana
ccaaacuaauaccuauucuguuuaguacuuc

SEQ ID NO: 383 - RNA, 31 nt, Arabidopsis thaliana
caggugcuuuuguugcguauaauguaaaucc

SEQ ID NO: 384 - RNA, 31 nt, Arabidopsis thaliana
cuuucaaacuaguacuuuuuguaaucgacuc

SEQ ID NO: 385 - RNA, 31 nt, Arabidopsis thaliana
aguuuugaaugacuuucuagucagaucguuc

SEQ ID NO: 386 - RNA, 31 nt, Arabidopsis thaliana
aucauuaugccuuugcaauguuacuugguuc

SEQ ID NO: 387 - RNA, 31 nt, Arabidopsis thaliana
uacuugguucaacucuauuugugaccuuuuc

SEQ ID NO: 388 - RNA, 31 nt, Arabidopsis thaliana
cuugguucaacucuauuugugaccuuuucuc

SEQ ID NO: 389 - RNA, 31 nt, Arabidopsis thaliana
ucuauuugugaccuuuucucguaugugggac

SEQ ID NO: 390 - RNA, 31 nt, Arabidopsis thaliana
acucucuaucuucuuggguagauaaucgauc

SEQ ID NO: 391 - RNA, 31 nt, Arabidopsis thaliana
augcuucuuggggcuucuuguucgauagccc

SEQ ID NO: 392 - RNA, 31 nt, Arabidopsis thaliana
cgaccguagugauguuaauugugguuacauc

SEQ ID NO: 393 - RNA, 31 nt, Arabidopsis thaliana
agcccucgauuuauguguuauuuauccauuc

SEQ ID NO: 394 - RNA, 31 nt, Arabidopsis thaliana
guuauuuauccauucuuacuuuuuuuaugcc

SEQ ID NO: 395 - RNA, 31 nt, Arabidopsis thaliana
uuaugccaauguuggugacuggagauaacuc

SEQ ID NO: 396 - RNA, 31 nt, Arabidopsis thaliana
uuacacgacuucaggcagauaaagcagcuac

SEQ ID NO: 397 - RNA, 31 nt, Arabidopsis thaliana
uaggugauuuuggauuagcucuugggauuuc

SEQ ID NO: 398 - RNA, 31 nt, Arabidopsis thaliana
gauuuuggauuagcucuugggauuucggguc

SEQ ID NO: 399 - RNA, 31 nt, Arabidopsis thaliana
caaacaguagacuuuucaaccauuuuugcuc

SEQ ID NO: 400 - RNA, 31 nt, Arabidopsis thaliana
acuuuucaaccauuuuugcucgugcuagugc

SEQ ID NO: 401 - RNA, 31 nt, Arabidopsis thaliana
cuuuucaaccauuuuugcucgugcuagugcc

SEQ ID NO: 402 - RNA, 31 nt, Arabidopsis thaliana
gugcuagugcccccagaaauucuuggauuuc

SEQ ID NO: 403 - RNA, 31 nt, Arabidopsis thaliana
aaugccauaagucuuauuuguauuuuacuuc

SEQ ID NO: 404 - RNA, 31 nt, Arabidopsis thaliana
gugcuguugggaaauccgcgcagauaggauc

SEQ ID NO: 405 - RNA, 31 nt, Arabidopsis thaliana
aauccgcgcagauaggaucgcauacuugguc

SEQ ID NO: 406 - RNA, 31 nt, Arabidopsis thaliana
cuauggagggucccacuccaguauccgcuuc

SEQ ID NO: 407 - RNA, 31 nt, Arabidopsis thaliana
auagcaaggugcuccccuuuauuugaauacc

SEQ ID NO: 408 - RNA, 31 nt, Arabidopsis thaliana
acccaccuacggcuuugauuguuauuacuuc

SEQ ID NO: 409 - RNA, 31 nt, Arabidopsis thaliana
cuuugauuguuauuacuucugcaggagcuac

SEQ ID NO: 410 - RNA, 31 nt, Arabidopsis thaliana
cauuccguuuuguuucccaucccagucuuuc

SEQ ID NO: 411 - RNA, 31 nt, Arabidopsis thaliana
uaggucucgacuucuucgcuaugaucuuccc

SEQ ID NO: 412 - RNA, 31 nt, Arabidopsis thaliana
gacuucuucgcuaugaucuucccaguaguuc

SEQ ID NO: 413 - RNA, 31 nt, Arabidopsis thaliana
caguaguucauauaggagcuauagccguuuc

SEQ ID NO: 414 - RNA, 31 nt, Arabidopsis thaliana
guaccaugauacuuucuguuuugucgagccc

SEQ ID NO: 415 - RNA, 31 nt, Arabidopsis thaliana
cauugggcaauuuacuuuauaccuacuauuc

SEQ ID NO: 416 - RNA, 31 nt, Arabidopsis thaliana
uauaccuacuauucugucugguuuuugguuc

SEQ ID NO: 417 - RNA, 31 nt, Arabidopsis thaliana
gcccugcuuuggucucugguuugaugguugc

SEQ ID NO: 418 - RNA, 31 nt, Arabidopsis thaliana
gcuaaaaauccgguacauuccguuuuguuuc

SEQ ID NO: 419 - RNA, 31 nt, Arabidopsis thaliana
cuaaaaauccgguacauuccguuuuguuucc

SEQ ID NO: 420 - RNA, 31 nt, Arabidopsis thaliana
auccgguacauuccguuuuguuucccauccc

SEQ ID NO: 421 - RNA, 31 nt, Arabidopsis thaliana
cuuucuggucaguaauggaagcaaucguccc

SEQ ID NO: 422 - RNA, 31 nt, Arabidopsis thaliana
gucaguaauggaagcaaucgucccuaccguc

SEQ ID NO: 423 - RNA, 31 nt, Arabidopsis thaliana
ccuaccgucguaaaauaagagcacccggcuc

SEQ ID NO: 424 - RNA, 31 nt, Arabidopsis thaliana
accgucguaaaauaagagcacccggcucugc

SEQ ID NO: 425 - RNA, 31 nt, Arabidopsis thaliana
guaaaauaagagcacccggcucugcccauuc

SEQ ID NO: 426 - RNA, 31 nt, Arabidopsis thaliana
ccggcucugcccauucacaaggacucgauuc

SEQ ID NO: 427 - RNA, 31 nt, Arabidopsis thaliana
gacucgauucuauguccaaacaucacaugcc

SEQ ID NO: 428 - RNA, 31 nt, Arabidopsis thaliana
guccaaacaucacaugccagcagaugugguc

SEQ ID NO: 429 - RNA, 31 nt, Arabidopsis thaliana
ugguggaacgugcggaaccacauauuggauc

SEQ ID NO: 430 - RNA, 31 nt, Arabidopsis thaliana
acaaaacuuaucuucaagcuuuaccuuauuc

SEQ ID NO: 431 - RNA, 31 nt, Arabidopsis thaliana
aucuucaagcuuuaccuuauucugaucguuc

SEQ ID NO: 432 - RNA, 31 nt, Arabidopsis thaliana
ucaagcuuuaccuuauucugaucguucagac

SEQ ID NO: 433 - RNA, 31 nt, Arabidopsis thaliana
cuuucccaugacgacuaggaaaaggcaaauc

SEQ ID NO: 434 - RNA, 31 nt, Arabidopsis thaliana
uauguuucuaugauggcccaagaacacgcuc

SEQ ID NO: 435 - RNA, 31 nt, Arabidopsis thaliana
cuaugauggcccaagaacacgcucauucuuc

SEQ ID NO: 436 - RNA, 31 nt, Arabidopsis thaliana
uuacgagcucaauauauacgaguguuauucc

SEQ ID NO: 437 - RNA, 31 nt, Arabidopsis thaliana
gaguguuauuccgugaaauaacucgaauuuc

SEQ ID NO: 438 - RNA, 31 nt, Arabidopsis thaliana
uccgugaaauaacucgaauuucaaaucauuc

SEQ ID NO: 439 - RNA, 31 nt, Arabidopsis thaliana
cuaggaaaaggcaaaucaaaaauuuuacuuc

SEQ ID NO: 440 - RNA, 31 nt, Arabidopsis thaliana
cuucucguaucgaugaauuagaagagauguc

SEQ ID NO: 441 - RNA, 31 nt, Arabidopsis thaliana
uggggauucagugguguaauguuaagagguc

SEQ ID NO: 442 - RNA, 31 nt, Arabidopsis thaliana
uguuaagagguccagggguaugcugggauuc

SEQ ID NO: 443 - RNA, 31 nt, Arabidopsis thaliana
gauucgcgaagagcagcaccuuacgauguuc

SEQ ID NO: 444 - RNA, 31 nt, Arabidopsis thaliana
gagcagcaccuuacgauguucaugaccaauc

SEQ ID NO: 445 - RNA, 31 nt, Arabidopsis thaliana
gcaccuuacgauguucaugaccaaucggauc

SEQ ID NO: 446 - RNA, 31 nt, Arabidopsis thaliana
cuugacguaccaguagguaccagaggagauc

SEQ ID NO: 447 - RNA, 31 nt, Arabidopsis thaliana
gaccucaacauccugcugcucaugguguuuc

SEQ ID NO: 448 - RNA, 31 nt, Arabidopsis thaliana
cagaggagaucgcuaugaucguuacuguauc

SEQ ID NO: 449 - RNA, 31 nt, Arabidopsis thaliana
agaucgcuaugaucguuacuguauccguauc

SEQ ID NO: 450 - RNA, 31 nt, Arabidopsis thaliana
gaugucgaaugaaacuauccauggaauccuc

SEQ ID NO: 451 - RNA, 31 nt, Arabidopsis thaliana
ccauuucgaacuuuauacagaagguuuuucc

SEQ ID NO: 452 - RNA, 31 nt, Arabidopsis thaliana
aauugcauaccuauacaaggguucaaguuuc

SEQ ID NO: 453 - RNA, 31 nt, Arabidopsis thaliana
caaguuucgaucgauauuugcggaguugauc

SEQ ID NO: 454 - RNA, 31 nt, Arabidopsis thaliana
accagugcagacgaaguaacacgaauaucuc

SEQ ID NO: 455 - RNA, 31 nt, Arabidopsis thaliana
ccgguaguaagucuauuuccaucagccggcc

SEQ ID NO: 456 - RNA, 31 nt, Arabidopsis thaliana
ucaucaaucauccggaucuacgccguauauc

SEQ ID NO: 457 - RNA, 31 nt, Arabidopsis thaliana
gguuucgagggucauccauuacgaaaagacc

SEQ ID NO: 458 - RNA, 31 nt, Arabidopsis thaliana
aaauggaaagaucggaacaugggaauagauc

SEQ ID NO: 459 - RNA, 31 nt, Arabidopsis thaliana
cuuggaaaaaaucguaguucagauucaaguc

SEQ ID NO: 460 - RNA, 31 nt, Arabidopsis thaliana; identical to SEQ ID NO: 459

SEQ ID NO: 461 - RNA, 31 nt, Arabidopsis thaliana
ugguuugacaugguuuacguguuacugguuc

SEQ ID NO: 462 - RNA, 31 nt, Arabidopsis thaliana
gguuugacaugguuuacguguuacugguucc

SEQ ID NO: 463 - RNA, 31 nt, Arabidopsis thaliana
cguguuacugguucccggaagaguuaauauc

SEQ ID NO: 464 - RNA, 31 nt, Arabidopsis thaliana
guuacugguucccggaagaguuaauaucucc

SEQ ID NO: 465 - RNA, 31 nt, Arabidopsis thaliana
ucccggaagaguuaauaucuccauuagcguc

SEQ ID NO: 466 - RNA, 31 nt, Arabidopsis thaliana
ggaagaguuaauaucuccauuagcgucaccc

SEQ ID NO: 467 - RNA, 31 nt, Arabidopsis thaliana
cgucacccuuucuuacccugccuuuugacuc

SEQ ID NO: 468 - RNA, 31 nt, Arabidopsis thaliana
ggagaacaaaggacgaaauacaaucgauucc

SEQ ID NO: 469 - RNA, 31 nt, Arabidopsis thaliana
gaacaaaggacgaaauacaaucgauuccucc

SEQ ID NO: 470 - RNA, 31 nt, Arabidopsis thaliana
aauacaaucgauuccuccauuuaagugguuc

SEQ ID NO: 471 - RNA, 31 nt, Arabidopsis thaliana
uacaaucgauuccuccauuuaagugguucuc

SEQ ID NO: 472 - RNA, 31 nt, Arabidopsis thaliana
auuccuccauuuaagugguucucgcuucuuc

SEQ ID NO: 473 - RNA, 31 nt, Arabidopsis thaliana
ucucgcuucuucuuguuccuguuccuaacuc

SEQ ID NO: 474 - RNA, 31 nt, Arabidopsis thaliana
cucgcuucuucuuguuccuguuccuaacucc

SEQ ID NO: 475 - RNA, 31 nt, Arabidopsis thaliana
cgcuucuucuuguuccuguuccuaacuccuc

SEQ ID NO: 476 - RNA, 31 nt, Arabidopsis thaliana
uucuucuuguuccuguuccuaacuccucccc

SEQ ID NO: 477 - RNA, 31 nt, Arabidopsis thaliana
cccgggucguucccaauguuuggcacuuucc

SEQ ID NO: 478 - RNA, 31 nt, Arabidopsis thaliana
cuucgugggugcaacaucaacaaauucgcuc

SEQ ID NO: 479 - RNA, 31 nt, Arabidopsis thaliana
augaucaaguuacaaccuaagaucuaugacc

SEQ ID NO: 480 - RNA, 31 nt, Arabidopsis thaliana
augaccauauuauguuaacuguucguauuuc

SEQ ID NO: 481 - RNA, 31 nt, Arabidopsis thaliana
auuauguuaacuguucguauuucguucauuc

SEQ ID NO: 482 - RNA, 31 nt, Arabidopsis thaliana
ucguauuucguucauuccaucgguaugcucc

SEQ ID NO: 483 - RNA, 31 nt, Arabidopsis thaliana
cccagguaccuguaauugugaucuguuugcc

SEQ ID NO: 484 - RNA, 31 nt, Arabidopsis thaliana
guaccuguaauugugaucuguuugccagaac

SEQ ID NO: 485 - RNA, 31 nt, Arabidopsis thaliana
uaccuguaauugugaucuguuugccagaacc

SEQ ID NO: 486 - RNA, 31 nt, Arabidopsis thaliana
uauauauauccuaugaauuuaauuucgcauc

SEQ ID NO: 487 - RNA, 31 nt, Arabidopsis thaliana
acgaacaaucgucguuuuuugaugguuuuuc

SEQ ID NO: 488 - RNA, 31 nt, Arabidopsis thaliana
aaucgucguuuuuugaugguuuuuccgcuuc

SEQ ID NO: 489 - RNA, 31 nt, Arabidopsis thaliana
ugguuuuuccgcuucucacagcugcucuuuc

SEQ ID NO: 490 - RNA, 31 nt, Arabidopsis thaliana
gguuuuuccgcuucucacagcugcucuuucc

SEQ ID NO: 491 - RNA, 31 nt, Arabidopsis thaliana
uuccacaccuccggauaucuggugccaaauc

SEQ ID NO: 492 - RNA, 31 nt, Arabidopsis thaliana
ccuccggauaucuggugccaaaucgucgccc

SEQ ID NO: 493 - RNA, 31 nt, Arabidopsis thaliana
ggauaucuggugccaaaucgucgcccguuuc

SEQ ID NO: 494 - RNA, 31 nt, Arabidopsis thaliana
ugauaauagaguuggcuauuuuuguggcauc

SEQ ID NO: 495 - RNA, 31 nt, Arabidopsis thaliana
auucuaggagaaguucgaauccguuccguuc

SEQ ID NO: 496 - RNA, 31 nt, Arabidopsis thaliana
ccuuugcacgagucagaaaccgauguauuuc

SEQ ID NO: 497 - RNA, 31 nt, Arabidopsis thaliana
aaagcuuuauaaagccuuuuguaaagauccc

SEQ ID NO: 498 - RNA, 31 nt, Arabidopsis thaliana
guacaaaacuggguuuuggaagauauggcac

SEQ ID NO: 499 - RNA, 31 nt, Arabidopsis thaliana
agauauggcacuaaaaguuguaaagcugguc

SEQ ID NO: 500 - RNA, 31 nt, Arabidopsis thaliana
uauuuaaccauaaaaucgauuaugcuccugc

SEQ ID NO: 501 - RNA, 31 nt, Arabidopsis thaliana
auaaaaucgauuaugcuccugcggaaguauc

SEQ ID NO: 502 - RNA, 31 nt, Arabidopsis thaliana
ggauugcucguguguccacgggacaaauccc

SEQ ID NO: 503 - RNA, 31 nt, Arabidopsis thaliana
gacaagccgcuacauuagcggcucauaaacc

SEQ ID NO: 504 - RNA, 31 nt, Arabidopsis thaliana
ccgcuacauuagcggcucauaaaccauguuc

SEQ ID NO: 505 - RNA, 31 nt, Arabidopsis thaliana
cugcggaaguaucuacucguuacggaaucuc

SEQ ID NO: 506 - RNA, 31 nt, Arabidopsis thaliana
augacccuaaucguucuucucagaucgcucc

SEQ ID NO: 507 - RNA, 31 nt, Arabidopsis thaliana
aaguucgcuccgccgcgcaagauccucgaac

SEQ ID NO: 508 - RNA, 31 nt, Arabidopsis thaliana
aacgcauagcauucucugggcacauaggauc

SEQ ID NO: 509 - RNA, 31 nt, Arabidopsis thaliana
aaaaauggaaaauuggcuauggagauuccgc

SEQ ID NO: 510 - RNA, 31 nt, Arabidopsis thaliana
cucuccgagggcauggaaugucuaauuuuuc

SEQ ID NO: 511 - RNA, 31 nt, Arabidopsis thaliana
auggaaugucuaauuuuucggucagaaucuc

SEQ ID NO: 512 - RNA, 31 nt, Arabidopsis thaliana
uuccacucaauuuucauuacgaagauguauc

SEQ ID NO: 513 - RNA, 31 nt, Arabidopsis thaliana
uucauuacgaagauguaucacgucaagaucc

SEQ ID NO: 514 - RNA, 31 nt, Arabidopsis thaliana
cuucggccaacacacaagaugagacuuuacc

SEQ ID NO: 515 - RNA, 31 nt, Arabidopsis thaliana
gauguaucacgucaagauccguugcucaaac

SEQ ID NO: 516 - RNA, 31 nt, Arabidopsis thaliana
auguaucacgucaagauccguugcucaaacc

SEQ ID NO: 517 - RNA, 31 nt, Arabidopsis thaliana
ucacgucaagauccguugcucaaaccgaauc

SEQ ID NO: 518 - RNA, 31 nt, Arabidopsis thaliana
aucacgccaacguuauggaaguuccuggauc

SEQ ID NO: 519 - RNA, 31 nt, Arabidopsis thaliana
auaaauguccccagaaaacaggaguaugccc

SEQ ID NO: 520 - RNA, 31 nt, Arabidopsis thaliana
cgagaacaccgaaaaaaccuaauuccgcucc

SEQ ID NO: 521 - RNA, 31 nt, Arabidopsis thaliana
cgguugagcaaucgacaugauauauuugcuc

SEQ ID NO: 522 - RNA, 31 nt, Arabidopsis thaliana
uugcucacaucccgggcgaaggucauaauuc

SEQ ID NO: 523 - RNA, 31 nt, Arabidopsis thaliana
uguuaauaagaggagguagagugaaagauuc

SEQ ID NO: 524 - RNA, 31 nt, Arabidopsis thaliana
guagagugaaagauucgccagguguaaaauc

SEQ ID NO: 525 - RNA, 31 nt, Arabidopsis thaliana
uagagugaaagauucgccagguguaaaaucc

SEQ ID NO: 526 - RNA, 31 nt, Arabidopsis thaliana
ggaccguacucgagcuuuggauaaauguccc

SEQ ID NO: 527 - RNA, 31 nt, Arabidopsis thaliana
caaucaauuaagggucaaauguuggaaccuc

SEQ ID NO: 528 - RNA, 31 nt, Arabidopsis thaliana
gaaagagaggaauuccguacagguacaacuc

SEQ ID NO: 529 - RNA, 31 nt, Arabidopsis thaliana
guaucaagaugucaaucugagaucuuauuuc

SEQ ID NO: 530 - RNA, 31 nt, Arabidopsis thaliana
guacagguacaacucuuauuuuuacgaaguc

SEQ ID NO: 531 - RNA, 31 nt, Arabidopsis thaliana
uuuuuacgaagucaaaaaaaugcgaucuuuc

SEQ ID NO: 532 - RNA, 31 nt, Arabidopsis thaliana
gucagucaaaauaaaaucuguuuaucaaagc

SEQ ID NO: 533 - RNA, 31 nt, Arabidopsis thaliana
aaaauaaaaucuguuuaucaaagcgcuucuc

SEQ ID NO: 534 - RNA, 31 nt, Arabidopsis thaliana
aaauaaaaucuguuuaucaaagcgcuucucc

SEQ ID NO: 535 - RNA, 31 nt, Arabidopsis thaliana
agggguggagggaauccguauauguuuuucc

SEQ ID NO: 536 - RNA, 31 nt, Arabidopsis thaliana
aaacuaaaugcuauaagcauagaaaaacuuc

SEQ ID NO: 537 - RNA, 31 nt, Arabidopsis thaliana
acuaaaugcuauaagcauagaaaaacuucuc

SEQ ID NO: 538 - RNA, 31 nt, Arabidopsis thaliana; identical to SEQ ID NO: 500

SEQ ID NO: 539 - RNA, 31 nt, Arabidopsis thaliana; identical to SEQ ID NO: 501

SEQ ID NO: 540 - RNA, 31 nt, Arabidopsis thaliana; identical to SEQ ID NO: 505

SEQ ID NO: 541 - RNA, 31 nt, Arabidopsis thaliana
uucggcuuucgucucgguagguguauuauuc

SEQ ID NO: 542 - RNA, 31 nt, Arabidopsis thaliana
accgauuacccucgauaaagaagaaucuuuc

SEQ ID NO: 543 - RNA, 31 nt, Arabidopsis thaliana
uacccucgauaaagaagaaucuuucuaaauc

SEQ ID NO: 544 - RNA, 31 nt, Arabidopsis thaliana
agcguuccugauagaaaaugacgacuccuuc

SEQ ID NO: 545 - RNA, 31 nt, Arabidopsis thaliana; identical to SEQ ID NO: 459

SEQ ID NO: 546 - RNA, 31 nt, Arabidopsis thaliana
guucucguaucgcuuuuuuuguagaaagcuc

SEQ ID NO: 547 - RNA, 31 nt, Arabidopsis thaliana
cauaucccucacgacauaagauuaaaagauc

SEQ ID NO: 548 - RNA, 31 nt, Arabidopsis thaliana
auaucccucacgacauaagauuaaaagaucc

SEQ ID NO: 549 - RNA, 31 nt, Arabidopsis thaliana
acgacauaagauuaaaagauccaaaccuucc

SEQ ID NO: 550 - RNA, 31 nt, Arabidopsis thaliana
auaagauuaaaagauccaaaccuuccucuuc

SEQ ID NO: 551 - RNA, 31 nt, Arabidopsis thaliana
aagagaucuauuaagaagagaaagauuuauc

SEQ ID NO: 552 - RNA, 31 nt, Arabidopsis thaliana
uauauacaauuacaaacuacacgaaaguugc

SEQ ID NO: 553 - RNA, 31 nt, Arabidopsis thaliana
auacaauuacaaacuacacgaaaguugcccc

SEQ ID NO: 554 - RNA, 31 nt, Arabidopsis thaliana
uuacaaacuacacgaaaguugccccuuuuuc

SEQ ID NO: 555 - RNA, 31 nt, Arabidopsis thaliana
gaacaaaacgaacuucauauaucccuuuucc

SEQ ID NO: 556 - RNA, 31 nt, Arabidopsis thaliana
gaacuucauauaucccuuuuccacucaaucc

SEQ ID NO: 557 - RNA, 31 nt, Arabidopsis thaliana
ucaauccagaaacaagauuugacguuauucc

SEQ ID NO: 558 - RNA, 31 nt, Arabidopsis thaliana
acaagauuugacguuauuccgcuucgucucc

SEQ ID NO: 559 - RNA, 31 nt, Arabidopsis thaliana
uucuugaaacuauuccucaagcaaggcagcc

SEQ ID NO: 560 - RNA, 31 nt, Arabidopsis thaliana
aaauaaggagaucuuucuauaaagaaauuuc

SEQ ID NO: 561 - RNA, 31 nt, Arabidopsis thaliana
cauuaagauuucaaacuugucgucuacuuuc

SEQ ID NO: 562 - RNA, 31 nt, Arabidopsis thaliana
caaacuugucgucuacuuucaggaaauguuc

SEQ ID NO: 563 - RNA, 31 nt, Arabidopsis thaliana
ucaaaaggaucgaacuaccuacucauuauuc

SEQ ID NO: 564 - RNA, 31 nt, Arabidopsis thaliana
gaacuaccuacucauuauucggagguuaauc

SEQ ID NO: 565 - RNA, 31 nt, Arabidopsis thaliana
uuaaucauagaacaccaaaagcugugguauc

SEQ ID NO: 566 - RNA, 31 nt, Arabidopsis thaliana
uaagcuauaggauaagcuuagagaaauguuc

SEQ ID NO: 567 - DNA, 32 bp, Artificial Sequence
  Enko_B-F primer
cgcgaattcagcggagagagttgcgaagcagg

SEQ ID NO: 568 - DNA, 31 bp, Artificial Sequence
  Enko_B-R primer
cgcgtcgactcatcccccaaatgatagatcc

SEQ ID NO: 569 - DNA, 32 bp, Artificial Sequence; identical to SEQ ID NO: 567
  Kosena_B-F primer

SEQ ID NO: 570 - DNA, 31 bp, Artificial Sequence; identical to SEQ ID NO: 568
  Kosena_B-R primer

SEQ ID NO: 571 - DNA, 38 bp, Artificial Sequence
  Enko A-F primer
cgcgaattcagcagggatggagagagtggcgaagcagg

SEQ ID NO: 572 - DNA, 54 bp, Artificial Sequence
  Enko A-R primer
cgcgtcgacttcatcctccaactgatatcccacactcatctgcagatcctcaag

SEQ ID NO: 573 - DNA, 2064 bp, Raphanus sativus
atgttggctagggtttgtggattcaagtgttcttcttctcctgctgagtctgcggctagattgttctgtacgagatcgattcgtgatactctggccaaggcaagcggagagagttgcgaagcaggttttggaggagagagtttgaagctgcaaagtgggtttcatgaaatcaaaggtttagaggatgcgattgatttgttcagtgacatgcttcgatctcgtcctttaccttctgtggttgatttctgtaaattgatgggtgtggtggtgagaatggaacgcccggatcttgtgatttctctctatcagaagatggaaaggaaacagattcgatgtgatatatacagcttcaatattctgataaaatgtttctgcagctgctctaagctcccctttgctttgtctacatttggtaagatcaccaagcttggactccaccctgatgttgttaccttcaccaccctgctccatggattatgtgtggaagatagggtttctgaagccttggatttttttcatcaaatgtttgaaacgacatgtaggcccaatgtcgtaaccttcaccactttgatgaacggtctttgccgcgagggtagaattgtcgaagccgtagctctgcttgatcggatgatggaagatggtctccagcctacccagattacttatggaacaatcgtagatgggatgtgtaagaagggagatactgtgtctgcactgaatctgctgaggaagatggaggaggtgagccacatcatacccaatgttgtaatctatagtgcaatcattgatagcctttgtaaagacggacgtcatagcgatgcacaaaatcttttcactgaaatgcaagagaaaggaatctttcccgatttatttacctacaacagtatgatagttggtttttgtagctctggtagatggagcgacgcggagcagttgttgcaagaaatgttagaaaggaagatcagccctgatgttgtaacttataatgctttgatcaatgcatttgtcaaggaaggcaagttctttgaggctgaagaattatacgatgagatgcttccaaggggtataatccctaatacaatcacatatagttcaatgatcgatggattttgcaaacagaatcgtcttgatgctgctgagcacatgttttatttgatggctaccaagggctgctctcccaacctaatcactttcaatactctcatagacggatattgtggggctaagaggatagatgatggaatggaacttctccatgagatgactgaaacaggattagttgctgacacaactacttacaacactcttattcacgggttctatctggtgggcgatcttaatgctgctctagaccttttacaagagatgatctctagtggtttgtgccctgatatcgttacttgtgacactttgctggatggtctctgcgataatgggaaactaaaagatgcattggaaatgtttaaggttatgcagaagagtaagaaggatcttgatgctagtcaccccttcaatggtgtggaacctgatgttcaaacttacaatatattgatcagcggcttgatcaatgaagggaagtttttagaggccgaggaattatacgaggagatgccccacaggggtatagtcccagatactatcacctatagctcaatgatcgatggattatgcaagcagagccgcctagatgaggctacacaaatgtttgattcgatgggtagcaagagcttctctccaaacgtagtgacctttactacactcattaatggctactgtaaggcaggaagggttgatgatgggctggagcttttctgcgagatgggtcgaagagggatagttgctaacgcaattacttacatcactttgatttgtggttttcgtaaagtgggtaatattaatggggctctagacattttccaggagatgatttcaagtggtgtgtatcctgataccattaccatccgcaatatgctgactggtttatggagtaaagaggaactaaaaagggcagtggcaatgcttgagaaactgcagatgagtatggatctatcatttgggggatga

SEQ ID NO: 574 - DNA, 2064 bp, Raphanus sativus
atgttggctagggtttgtggattcaagtgttcttcttctcctgctgagtctgcggctagattgttctgtacgagatcgattcgtgatactctggccaaggcaagcggagagagttgcgaagcaggttttggaggagagagtttgaagctgcaaagtgggtttcatgaaatcaaaggtttagaggatgcgattgatttgttcagtgacatgcttcgatctcgtcctttaccttctgtggttgatttctgtaaattgatgggtgtggtggtgagaatggaacgcccggatcttgtgatttctctctatcagaagatggaaaggaaacagattcgatgtgatatatacagcttcaccattctgataaaatgtttctgcagctgctctaagctcccctttgctttgtctacatttggtaagatcaccaagcttggactccaccctgatgttgttaccttcaacaccctgctccacggattgtgcgtggaagatagggtttctgaagctttgaatttgtttcatcaaatgtttgaaacgacatgtaggcccaatgtcgtaaccttcaccactttgatgaacggtctttgccgcgagggtagaattgtcgaagccgtagctctgcttgatcggatgatggaagatggtctccagcctacccagattacttatggaacaatcgtagatgggatgtgtaagaagggagatactgtgtctgcattgaatcttctgaggaagatggaggaggtgagccacatcatacccaatgttgtaatctatagtgcaatcattgatagcctttgtaaagacggacgtcatagcgatgcacaaaatcttttcactgaaatgcaagagaaaggaatctttcccgatttatttacctacaacagtatgatagttggtttttgtagctctggtagatggagcgacgcggagcagttgttgcaagaaatgttagaaaggaagatcagccctgatgttgtaacttataatgctttgatcaatgcatttgtcaaggaaggcaagttctttgaggctgaagaattatacgatgagatgcttccaaggggtataatccctaatacaatcacatatagttcaatgatcgatggattttgcaaacagaatcgtcttgatgctgctgagcacatgttttatttgatggctaccaagggctgctctcccaacctaatcactttcaatactctcatagacggatattgtggggctaagaggatagatgatggaatggaacttctccatgagatgactgaaacaggattagttgctgacacaactacttacaacactcttattcacgggttctatctggtgggcgatcttaatgctgctctagaccttttacaagagatgatctctagtggtttgtgccctgatatcgttacttgtgacactttgctggatggtctctgcgataatgggaaactaaaagatgcattggaaatgtttaaggttatgcagaagagtaagaaggatcttgatgctagtcaccccttcaatggtgtggaacctgatgttcaaacttacaatatattgatcagcggcttgatcaatgaagggaagtttttagaggccgaggaattatacgaggagatgccccacaggggtatagtcccagatactatcacctatagctcaatgatcgatggattatgcaagcagagccgcctagatgaggctacacaaatgtttgattcgatgggtagcaagagcttctctccaaacgtagtgacctttactacactcattaatggctactgtaaggcaggaagggttgatgatgggctggagcttttctgcgagatgggtcgaagagggatagttgctaacgcaattacttacatcactttgatttgtggttttcgtaaagtgggtaatattaatggggctctagacattttccaggagatgatttcaagtggtgtgtatcctgataccattaccatccgcaatatgctgactggtttatggagtaaagaggaactaaaaagggcagtggcaatgcttgagaaactgcagatgagtatggatctatcatttgggggatga

SEQ ID NO: 575 - DNA, 2061 bp, Raphanus sativus
atgttggctagggtttgcagattcgagtcttcctcttcgtcttctgtgtctgcggctagatttttctgtacgggatcgattcgtcatgctctggccgagaaaagcagggatggagagagtggcgaagcaggttttagaggagagagtttgaaactgcgaagtggatcttatgaaatcaaagggttagaggatgcgattgatttgttcagtgacatgcttcgatctcgtcctttaccttctgtgattgatttcaacaagctaatgggtgcggtggtgagaatggaacgcccggatcttgtgatttctctctatcaaaagatggaaaggaaacagattcgatgtgatatatacagcttcaccattctgataaaatgtttctgcagttgctctaagctcccctttgctttgtctacatttggtaagctcaccaagcttggactccaccctgatgttgttaccttcaccaccctgctccacggattatgtcttgatcacagggtttctgaagccttggatttgtttcatcaaatttgtagaccagatgtcctaacgttcaccacgctgatgaatggtctttgccgcgagggtcgagttgtcgaagccgtagctctgcttgatcggatggtggaaaatggtctccagcctgaccagattacttacggaacatttgtagatgggatgtgtaagatgggcgacactgtgtctgcattgaatcttctgaggaagatggaggagataagccacatcaaacccaatgtggttatctatagtgccatcattgatggcctttgtaaagatggacgccatagcgattctcataatcttttcattgaaatgcaagacaagggaatctttccaaatatagttacctacaactgtatgatcggtggattttgcatctctggtagatggagtgcagcccagcggttgttgcaagaaatgttagaaaggaagatcagccctaatgttgtaacttataatgctttgatcaatgcatttgtcaaggaaggcaagttcttcgaggctgcagaattatacgatgagatgcttccaaggggtatcattcctaatacaatcacatataattcaatgatcgatgggttttgcaaacaggatcgtcttgatgctgctgaggacatgttttatttgatggctaccaagggctgctctccggacgtattcactttcactactctcatagacggatattgtggggctaagaggatagatgatggaatggaacttctccatgagatgcctagaagaggattagttgctaacacagttacttacaacactcttattcacgggttctgtctggtgggcgatcttaatgctgctctagacctttcacagcagatgatttctagtggtgtgtgccctgatatcgttacttgtaacactttgctggacggtctctgcgataatgggaaactaaaagatgcattggaaatgtttaaggctatgcagaagagtaagatggatcttgatgctagtcaccccttcaatggtgtggaacctgatgttctaacttacaatatattgatctgcggcttgatcaatgaagggaagtttttagaggccgaggaattatacgaggagatgccacacagaggtatagtcccagatactatcacctatagctcaatgatcgatggactatgcaagcagagccgcctagatgaggctacacaaatgtttgtttcgatgggtagcaagagcttctctcccaacgtagtgacatttaacacactcattaatggctactgtaaggcaggaagggttgatgatgggctggagcttttctgcgagatgggtcgaagagggatagttgctgatgcaattatttacatcactttgatttatggttttcgtaaagtgggtaatattaatggggctctagacattttccaggagatgatttcaagtggtgtgtatcctgataccattactatccgcaatatgctgactggtttttggagtaaagaggaactagaaagggcagtggcaatgcttgaggatctgcagatgagtgtggggtatcagttggaggatgaatga

SEQ ID NO: 576 - protein, 687 aa, Raphanus sativus
MLARVCGFKCSSSPAESAARLFCTRSIRDTLAKASGESCEAGFGGESLKLQSGFHEIKGLEDAIDLFSDMLRSRPLPSVVDFCKLMGVVVRMERPDLVISLYQKMERKQIRCDIYSFNILIKCFCSCSKLPFALSTFGKITKLGLHPDVVTFTTLLHGLCVEDRVSEALDFFHQMFETTCRPNVVTFTTLMNGLCREGRIVEAVALLDRMMEDGLQPTQITYGTIVDGMCKKGDTVSALNLLRKMEEVSHIIPNVVIYSAIIDSLCKDGRHSDAQNLFTEMQEKGIFPDLFTYNSMIVGFCSSGRWSDAEQLLQEMLERKISPDVVTYNALINAFVKEGKFFEAEELYDEMLPRGIIPNTITYSSMIDGFCKQNRLDAAEHMFYLMATKGCSPNLITFNTLIDGYCGAKRIDDGMELLHEMTETGLVADTTTYNTLIHGFYLVGDLNAALDLLQEMISSGLCPDIVTCDTLLDGLCDNGKLKDALEMFKVMQKSKKDLDASHPFNGVEPDVQTYNILISGLINEGKFLEAEELYEEMPHRGIVPDTITYSSMIDGLCKQSRLDEATQMFDSMGSKSFSPNVVTFTTLINGYCKAGRVDDGLELFCEMGRRGIVANAITYITLICGFRKVGNINGALDIFQEMISSGVYPDTITIRNMLTGLWSKEELKRAVAMLEKLQMSMDLSFGG

SEQ ID NO: 577 - protein, 687 aa, Raphanus sativus
MLARVCGFKCSSSPAESAARLFCTRSIRDTLAKASGESCEAGFGGESLKLQSGFHEIKGLEDAIDLFSDMLRSRPLPSVVDFCKLMGVVVRMERPDLVISLYQKMERKQIRCDIYSFTILIKCFCSCSKLPFALSTFGKITKLGLHPDVVTFNTLLHGLCVEDRVSEALNLFHQMFETTCRPNVVTFTTLMNGLCREGRIVEAVALLDRMMEDGLQPTQITYGTIVDGMCKKGDTVSALNLLRKMEEVSHIIPNVVIYSAIIDSLCKDGRHSDAQNLFTEMQEKGIFPDLFTYNSMIVGFCSSGRWSDAEQLLQEMLERKISPDVVTYNALINAFVKEGKFFEAEELYDEMLPRGIIPNTITYSSMIDGFCKQNRLDAAEHMFYLMATKGCSPNLITFNTLIDGYCGAKRIDDGMELLHEMTETGLVADTTTYNTLIHGFYLVGDLNAALDLLQEMISSGLCPDIVTCDTLLDGLCDNGKLKDALEMFKVMQKSKKDLDASHPFNGVEPDVQTYNILISGLINEGKFLEAEELYEEMPHRGIVPDTITYSSMIDGLCKQSRLDEATQMFDSMGSKSFSPNVVTFTTLINGYCKAGRVDDGLELFCEMGRRGIVANAITYITLICGFRKVGNINGALDIFQEMISSGVYPDTITIRNMLTGLWSKEELKRAVAMLEKLQMSMDLSFGG

SEQ ID NO: 578 - protein, 686 aa, Raphanus sativus
MLARVCRFESSSSSSVSAARFFCTGSIRHALAEKSRDGESGEAGFRGESLKLRSGSYEIKGLEDAIDLFSDMLRSRPLPSVIDFNKLMGAVVRMERPDLVISLYQKMERKQIRCDIYSFTILIKCFCSCSKLPFALSTFGKLTKLGLHPDVVTFTTLLHGLCLDHRVSEALDLFHQICRPDVLTFTTLMNGLCREGRVVEAVALLDRMVENGLQPDQITYGTFVDGMCKMGDTVSALNLLRKMEEISHIKPNVVIYSAIIDGLCKDGRHSDSHNLFIEMQDKGIFPNIVTYNCMIGGFCISGRWSAAQRLLQEMLERKISPNVVTYNALINAFVKEGKFFEAAELYDEMLPRGIIPNTITYNSMIDGFCKQDRLDAAEDMFYLMATKGCSPDVFTFTTLIDGYCGAKRIDDGMELLHEMPRRGLVANTVTYNTLIHGFCLVGDLNAALDLSQQMISSGVCPDIVTCNTLLDGLCDNGKLKDALEMFKAMQKSKMDLDASHPFNGVEPDVLTYNILICGLINEGKFLEAEELYEEMPHRGIVPDTITYSSMIDGLCKQSRLDEATQMFVSMGSKSFSPNVVTFNTLINGYCKAGRVDDGLELFCEMGRRGIVADAIIYITLIYGFRKVGNINGALDIFQEMISSGVYPDTITIRNMLTGFWSKEELERAVAMLEDLQMSVGYQLEDE

SEQ ID NO: 579 - DNA, 41 bp, Artificial Sequence
  A-F primer primer
aatacgactcactatagaagaagaagctgctttgtggagtg

SEQ ID NO: 580 - DNA, 24 bp, Artificial Sequence
  A-R primer primer
tgcatttatatgctgaagaaaagc

SEQ ID NO: 581 - DNA, 48 bp, Artificial Sequence
  B-F primer primer
tagataatacgactcactatagggatgattacctttttcgaaaaattg

SEQ ID NO: 582 - DNA, 38 bp, Artificial Sequence
  B-R primer primer
aaaccagcttagccaaatatgggccattagcaaataag

SEQ ID NO: 583 - DNA, 42 bp, Artificial Sequence
  C-F primer primer
aatacgactcactatagtatttggctaagctggttttctaac

SEQ ID NO: 584 - DNA, 27 bp, Artificial Sequence
  C-R primer primer
gacacctagccacccatactgaaattc

SEQ ID NO: 585 - protein, 667 aa, Raphanus sativus
MLARVCRFESSSSVPAARLFCTRSIRHTLAKKSSGKAGGFGGERLKLQSGFHEIKGLDDAIDLFGYMVRSRPLPCVIDFCKLLGVVVRMERPDVVISLHRKMEMRRIPCNIYSFTILIKCFCSCSKLPFALSTFGKITKLGFHPSLVTFSTLLHGLCVEDRVSEALHFFHQICKPNVIAFTTLMNGLCREGRVVEAVALLDRMVEDGLQPNQITYGTIVDGMCKMGDTVSALNLLRKMEEVSRIKPNVVIYSAIIDGLWKDGRQTDAQNLFSEMQEKGISPNLFTYNCMINGFCSSGRWSEAQRLLREMFERKMSPDVVTFSVLINALVKEGKFFEAEELYNEMLPRGIIPNTITYNSMIDGFSKQNRLDAAERMFYLMATKGCSPDVITFSILIDGYCGAKRVDDGMKLLHEMSRRGLVANTITYTTLIHGFCQLGNLNAALDLLQEMISSGVCPNVVTCNTLLDGLCNNGKLKDALEMFKVMQKSKMDLDASHPFNDVEPDVQTYNILICGLINEGKFSEAEELYEEMPHRGLVPDTITYNSVIDGLCKQSRLDEATQMFDSMGSKGFSPDVVTFTTLINGYCKVGRVGDGLEVFCEMGRRGIVANAITYRTLIHGFCQVGNINGALDIFQEMISSGVYPDTITIRNMLTGLWSKEELKRAVQCL

SEQ ID NO: 586 - protein, 683 aa, Raphanus sativus
MLARVCRFESSSSSSVSAARFFCTGSIRHALAEKSRDGESGEAGFRGESLKLRSGSYEIKGLEDAIDLFSDMLRSRPLPSVIDFNKLMGAVVRMERPDLVISLYQKMERKQIRCDIYSFTILIKCFCSCSKLPFALSTFGKLTKLGLHPDVVTFTTLLHGLCLDHRVSEALDLFHQICRPDVLTFTTLMNGLCREGRVVEAVALLDRMVENGLQPDQITYGTFVDGMCKMGDTVSALNLLRKMEEISHIKPNVVIYSAIIDGLCKDGRHSDSHNLFIEMQDKGIFPNIVTYNCMIGGFCISGRWSAAQRLLQEMLERKISPNVVTYNALINAFVKEGKFFEAAELYDEMLPRGIIPNTITYNSMIDGFCKQDRLDAAEDMFYLMATKGCSPDVFTFTTLIDGYCGAKRIDDGMELLHEMPRRGLVANTVTYNTLIHGFCLVGDLNAALDLSQQMISSGVCPDIVTCNTLLDGLCDNGKLKDALEMFKAMQKSKMDLDASHPFNGVEPDVLTYNILICGLINEGKFLEAEELYEEMPHRGIVPDTITYSSMIDGLCKQSRLDEATQMFVSMGSKSFSPNVVTFNTLINGYCKAGRVDDGLELFCEMGRRGIVADAIIYITLIYGFRKVGNINGALDIFQEMISSGVYPDTITIRNMLTGFWSKEELERAVAMLEDLQRYQLEDE

SEQ ID NO: 587 - protein, 687 aa, Raphanus sativus
MLARVCGFKCSSSPAESAARLFCTRSIRDTLAKASGESCEAGFGGESLKLQSGFHEIKGLEDAIDLFSDMLRSRPLPSVVDFCKLMGVVVRMKRPDVVISLHKKVEMRRIPCDAYSFNILIKCFCSCSKLPFALSTFGKITKLGLHPDVVTFTTLLHGLCVEDRVSEALNLFHQMFETTCRPNVVTFTTLMNGLCREGRIVEAVALLDRMMEDGLQPTQITYGTIVDGMCKKGDTVSALNLLRKMEEVSHIIPNVVIYSAIIDSLCKDGRHSDAQNLFTEMQEKGIFPDLFTYNSMIVGFCSSGRWSDAEQLLQEMLERKISPDVVTYNALINAFVKEGKFFEAEELYDEMLPRGIIPNTITYSSMIDGFCKQNRLDAAENMFYLMATKGCSPNLITFNTLIDGYCGAKRIDDGMELLHEMTETGLVADTTTYNTLIHGFCLVGDLNAALDLLQEMISSGLCPDIVTCDTLLDGLCDNGKLKDALEMFKVMQKSKKDLDASHPFNGVEPDVQTYNILISGLINEGKFLEAEELYEEMPHRGIVPDTITYSSMIDGLCKQSRLDEATQMFDSMGSKSFSPNVVTFTTLINGYCKAGRVDDGLELFCEMGRRGIVANAITYITLICGFRKVGNINGALDIFQEMISSGVYPDTITIRNMLTGLWSKEELKRAVAMLEKLQMSMDLSFGG

SEQ ID NO: 588 - protein, 690 aa, Raphanus sativus
MLARVCRFESSSSSSVSAARMFCTGSIRHALAKKGRDGESGEAGFGGESLKLRSGFHEIKGLEDAIDLFSDMLRSRPLPSVIDFNKLMGVVVRMERPDLVISLYQKMERKQIPCDVYSFNILIKCFCSCSKLPFALSTFGKITKLGLHPDVATFNTLLHGLCLDKRVSEALDLFHQMFETTCRPNIITFTTLMNGLCYEGRVVEAVALLDRMLEDGLQPDQITYGTIVDGMCKMGDTVSALNLLRKMEELSHIKPNVVIYSAIIDGLWKDGRHTDAQNLFSEMQEKGIFPNLFTYTCMINGFCDSGRWSEAQQLLQEMLVRKISPNVVTYSALINAFVKEGKFFEAEELYDEMLPRGIIPSTVTYSSMIDGFCKQNRLDAAEHMFYLMPTKGCSPNLITFNTLIAGYCRAKRVDDGMELLHEMTETGLVADTTTYNTLIHGFCLVDDLNAALDLSQQMISSGVCPDIVTCNTLLDGLCDNGKLKDALEMFKAMQKSKMDFDASHPFNDVEPDVLTYNILISGLINDGKFLGAEELYEEMPHRGIVPDTFTYNSMICGLCKQNRLDEAKQMSDSMGSKSFSPNVVTFNTLINGYCKAGRVDDGLELFCGMGQRGIVANAITYITLIHGFRKVDNINGALDIFQEMISSGVYPDTITIRNMLTGLWSKEELKRAVAMLEDLQMSVGYQLEDE

SEQ ID NO: 589 - protein, 690 aa, Raphanus sativus
MLARVCRFESSSSSSVSAARMFCTGSIRHALAKKGRDGESGEAGFGGESLKLRSGFHEIKGLEDAIDLFSDMLRSRPLPSVIDFNKLMGVVVRMERPDLVISLYQKMERKQIPCDVYSFNILIKCFCSCSKLPFALSTFGKITKLGLHPDVATFNTLLHGLCLDKRVSEALDLFHQMFETTCRPNIITFTTLMNGLCYEGRVVEAVALLDRMLEDGLQPDQITYGTIVDGMCKMGDTVSALNLLRKMEELSHIKPNVVIYSAIIDGLWKDGRHTDAQNLFSEMQEKGIFPNLFTYTCMINGFCDSGRWSEAQQLLQEMLVRKISPNVVTYSALINAFVKEGKFFEAEELYDEMLPRGIIPSTVTYSSMIDGFCKQNRLDAAEHMFYLMPTKGCSPNLITFNTLIAGYCRAKRVDDGMELLHEMTETGLVADTTTYNTLIHGFCLVDDLNAALDLSQQMISSGVCPDIVTCNTLLDGLCDNGKLKDALEMFKAMQKSKMDFDASHPFNDVEPDVLTYNILISGLINDGKFLGAEELYEEMPHRGIVPDTVTYNSVINGLCKQSRLNEAKQMSDSMGSRSFSPNVVTFNTLINGYCKAGRVDDGLELFCEMGRRGVVANAITYITLIHGFSKVGNINGALDIFQEMMASGVYPDTITIRNMLTGLWSKEEVKRAVAMLEDLQMSVGYQLEDE

SEQ ID NO: 590 - protein, 683 aa, Raphanus sativus
MLARVYRSGSSSSPAVSAARLFCTRSIRHALAKKSRDGESGFGGESLKLRSGFHEIKGLEDAIDLFGDMVRSRPLPSVIDFCKLMGVVVRMGRLDVVISLHRKMEMGRVPCNAYSFTILMKCFCSCSKLPFALSTFGKITKLGLHPDVVTFNTLLHGLCVEDRVSEALYLFHQMCKPNVVTFTTLMKGLCREGRVVEAVALLDRMVEDGLQPNQITYGTIVDGMCKMGDSVSALDLLRKMEEVSHIKPDVVIYSAIIDGLWKDGRHTDAQNLFSEMQDKRIFPDLFTYSCMIDGFCSSGRWSEAQQLLQEMLERKISPDVVTYNALINAFVKEGKFFEAEELYDEMLPRGIIPNTITYSSMIDGFCKQNRLDAAEHMFYLMATKGCSPDVFTFNTLIDGYCGAKRIDDGMELLHEMTEAGLVANTVTYTTLIHGFCQVGDLNSAQDLLQEMISSGVCPNVVTCNTLLDGLCDNGKLKDALKMFKAMQKSKKNFDASHPFNGVEPDVLTYNILICGLINEGKFIEAEELYEEMPHRGIVPDTITYSSMIDGLCKQSRLDEATQMSDSMGSKSFSPNVVTFNTLINGYCKAGRVDDGLELFCEMGRRGIVANAITYITLIYGSRKVGNINGALDIFQEMISSGVYPDTITIRNMLTGLWSKEELERAVAMLEVLQMSVGYQLEDE

SEQ ID NO: 591 - protein, 686 aa, Raphanus sativus
MLARVCRFESSSSSSVSAARLLCTRSIHLPLAEKSRDGENGEAGSGGESLKLQSGSYEIKGLEDAIDLFSDMLRSRPLPSVIDFNKLMGAVVRMERPDLVISLYQKMERKQIRCDIYSFTILIKCFCSCSKLPVALSTFGKLTKLGLHPDVVTFTTLLHGLCVEDRVSEALDLFHQMCKPNVVTFNTLMNGLCREGRVVEAVALLDQMVENGLQPDQITYGTIVDGMCKMGDTVSALNLLRKMEEVSHIIPNVVIYSAIIDGLCKDGRHSDAHNLFIEMQDKGIFPNIVTYNCMIGGFCISGRWSAAQRLLQEMLVRKISPNVVTYNALINAFVKEGKFFEAEELYDEMLPRGIIPNTITYNSMIDGFCKQNRLDAAEHMFYVMATKGCSPDVFTFNTLIDGYCGAKRIDDGMELLHEMTETGLVADTTTYNTLIHGFCLVGDLNAALDLLQEMVSSGVCPDIVTCNTLLDGLCDNGKLKDALEMFKAMQKSKMYIDASHPFNGVEPDVLTYNILICGLINEGKFLEAEELYEEMPHRGIVPDTITYSSMIDGLCKQSRLDEATQMFVSMGSKSFSPNVVTFNTLINGYCKAGRVDDGLELFCEMGRRGIVADAITYITLIYGFRKVGNINGALDIFQEMMASGVYPDTITIRNMLTGLWSKEELKRAVAMLEDLQMSVGYQLEDE